European Patent Application EP 4 737 581 A1, published May 6, 2026. Title: Novel spermidine and agmatine producing Bacillus strains. Applicant: Evonik Operations GmbH. The sequence listing filed with the application follows.

SEQUENCE LISTING (52 sequences)

SEQ ID NO: 1 - DNA, 1457 bp, Bacillus subtilis
  source 1..1457: mol_type = genomic DNA
gttagcggcggacgggtgagtaacacgtgggtaacctgcctgtaagactgggataactccgggaaaccggggctaataccggatggttgtttgaaccgcatggttcaaacataaaaggtggcttcggctaccacttacagatggacccgcggcgcattagctagttggtgaggtaatggctcaccaaggcaacgatgcgtagccgacctgagagggtgatcggccacactgggactgagacacggcccagactcctacgggaggcagcagtagggaatcttccgcaatggacgaaagtctgacggagcaacgccgcgtgagtgatgaaggttttcggatcgtaaagctctgttgttagggaagaacaagtaccgttcgaatagggcggtaccttgacggtacctaaccagaaagccacggctaactacgtgccagcagccgcggtaatacgtaggtggcaagcgttgtccggaattattgggcgtaaagggctcgcaggcggtttcttaagtctgatgtgaaagcccccggctcaaccggggagggtcattggaaactggggaacttgagtgcagaagaggagagtggaattccacgtgtagcggtgaaatgcgtagagatgtggaggaacaccagtggcgaaggcgactctctggtctgtaactgacgctgaggagcgaaagcgtggggagcgaacaggattagataccctggtagtccacgccgtaaacgatgagtgctaagtgttagggggtttccgccccttagtgctgcagctaacgcattaagcactccgcctggggagtacggtcgcaagactgaaactcaaaggaattgacgggggcccgcacaagcggtggagcatgtggtttaattcgaagcaacgcgaagaaccttaccaggtcttgacatcctctgacaatcctagagataggacgtccccttcgggggcagagtgacaggtggtgcatggttgtcgtcagctcgtgtcgtgagatgttgggttaagtcccgcaacgagcgcaacccttgatcttagttgccagcattcagttgggcactctaaggtgactgccggtgacaaaccggaggaaggtggggatgacgtcaaatcatcatgccccttatgacctgggctacacacgtgctacaatggacagaacaaagggcagcgaaaccgcgaggttaagccaatcccacaaatctgttctcagttcggatcgcagtctgcaactcgactgcgtgaagctggaatcgctagtaatcgcggatcagcatgccgcggtgaatacgttcccgggccttgtacacaccgcccgtcacaccacgagagtttgtaacacccgaagtcggtgaggtaaccttttaggagccagccgccgaaggtgggacagatgattggggtgaagtcgtaacaaggtagccgtatcggaaggtgcggctggatcacctccttt

SEQ ID NO: 2 - DNA, 1635 bp, Bacillus subtilis
  source 1..1635: mol_type = genomic DNA
atggcaaaagaaattaagtttagtgaagaagctcgccgcgcaatgcttcgcggtgtcgatgcacttgctgatgctgttaaagtaactttaggaccaaaaggacgcaacgtggttctagagaaaaaattcggttctccgttaatcacaaatgacggtgtaacaatcgctaaagaaatcgagctagaagacgcgtttgaaaacatgggtgctaagcttgttgctgaagtagccagcaaaacaaacgacgttgccggtgacggtacaacaactgcaacagttcttgcgcaagcaatgatccgtgaaggccttaaaaacgtaacagcaggcgctaaccctgtaggcgtgcgtaaagggatggaacaagctgtagcggttgcgatcgaaaacttaaaagaaatttctaagccaatcgaaggcaaagagtctatcgctcaggttgctgcgatctctgctgctgatgaggaagtcggaagccttatcgctgaagcaatggagcgcgtaggaaacgacggcgttatcacaatcgaagagtctaaaggcttcacaactgagcttgaagttgttgaaggtatgcaattcgaccgcggatatgcgtctccttacatggtaactgactctgataagatggaagcggttcttgacaatccttacatcttaatcacagacaaaaaaatcacaaacattcaagaaatccttcctgtgcttgagcaggttgttcagcaaggcaaaccattgcttctgatcgctgaggatgttgaaggcgaagcacttgcaacacttgttgtgaacaaacttcgcggcacattcaacgcagttgctgttaaagctcctggcttcggtgaccgccgtaaagcaatgcttgaagacatcgctgtccttactggcggagaagtcatcacagaagatcttggccttgacctgaaatctactcaaatcgctcaattgggacgcgcttctaaagttgtcgttactaaagaaaacacaacaatcgttgaaggcgctggcgaaacagacaaaatttctgcccgcgtgactcaaatccgcgctcaagtggaagaaacaacttctgaattcgacagagaaaaattacaagagcgtcttgcgaaacttgctggcggcgtagctgtcatcaaagtcggcgctgcgactgaaactgagctgaaagagcgtaaacttcgcatcgaagacgccttgaactcaactcgcgcagctgttgaagaaggcatcgtatccggtggcggtacagcgcttgtaaacgtatataacaaagtcgctgcagttgaagctgaaggcgatgctcaaacaggtatcaacatcgtgcttcgcgcgcttgaagagccaatccgtcaaatcgcacacaatgctggtcttgaaggatctgtcatcgttgagcgcctcaaaaacgaagaaatcggcgtaggcttcaacgctgcaactggcgaatgggtaaacatgatcgaaaaaggtatcgttgacccaactaaagttacacgctcagctcttcaaaacgctgcgtctgtagctgcaatgttcttaacaacagaagctgttgtcgctgacaagccagaagaaaacggtggcggcgcaggaatgcctgatatgggcggcatgggcggtatgggtggaatgatgtaa

SEQ ID NO: 3 - DNA, 1917 bp, Bacillus subtilis
  source 1..1917: mol_type = genomic DNA
atggaacagcagcaaaacagttatgatgaaaatcagatacaggtactagaaggattggaagctgttcgtaaaagaccggggatgtatatcggttcgacaaacagcaaaggccttcaccacctggtatgggaaattgtcgacaatagtattgacgaagccctcgccggttattgtacggatatcaatatccaaatcgaaaaagacaacagtatcacggttgtagataatggccgcggtattccagtcggtattcatgaaaaaatgggccgtcctgcggtagaagtcattatgacggtacttcatgccggaggaaaatttgacggaagcggctataaagtatccggaggattacacggtgtaggtgcgtctgtcgtaaacgcactatcaacagagcttgatgtgacggttcaccgtgacggtaaaattcaccgccaaacttataaacgcggagttccggttacagaccttgaaatcattggcgaaacggatcatacaggaacgacgacacattttgtcccggaccctgaaattttctcagaaacaaccgagtatgattatgatctgcttgccaaccgcgtacgtgaattagcctttttaacaaagggcgtaaacatcacgattgaggataaacgtgaaggacaagagcgcaaaaatgaataccattacgaaggcggaattaaaagttatgtagagtatttaaaccgctctaaagaggttgtccatgaagagccgatttacattgaaggcgaaaaggacggcattacggttgaagtggctttgcaatacaatgacagctacacaagcaacatttactcgtttacaaacaacattaacacgtacgaaggcggtacccatgaagctggcttcaaaacgggcctgactcgtgttatcaacgattacgccagaaaaaaagggcttattaaagaaaatgatccaaacctaagcggagatgacgtaagggaagggctgacagcgattatttcaatcaaacaccctgatccgcagtttgagggccaaacgaaaacaaagctgggcaactcagaagcacggacgatcaccgatacgttattttctacggcgatggaaacatttatgctggaaaatccagatgcagccaaaaaaattgtcgataaaggcttaatggcggcaagagcaagaatggctgcgaaaaaagcccgtgaactaacacgtcgtaagagtgctttggaaatttcaaacctgcccggtaagttagcggactgctcttcaaaagatccgagcatctccgagttatatatcgtagagggtgactctgccggaggatctgctaaacaaggacgcgacagacatttccaagccattttgccgcttagaggtaaaatcctaaacgttgaaaaggccagactggataaaatcctttctaacaacgaagttcgctctatgatcacagcgctcggcacaggtattggggaagacttcaaccttgagaaagcccgttaccacaaagttgtcattatgacagatgccgatgttgacggcgcgcacatcagaacacttctgttaacgttcttttacagatatatgcgccaaattatcgaaaatggctacgtgtacattgcgcagccgccgctctacaaggttcaacaggggaaacgcgttgaatatgcgtacaatgacaaggagcttgaagagctgttaaaaactcttcctcaaacgcctaagcctggactgcagcgttacaaaggtcttggtgaaatgaatgccacccagctatgggagacaaccatggatcctagttccagaacacttcttcaggtaactcttgaagatgcaatggatgcggacgagacttttgaaatgcttatgggcgacaaggtagaaccgcgccgaaacttcatagaagcgaatgcgagatacgttaaaaatcttgacatctaa

SEQ ID NO: 4 - DNA, 3582 bp, Bacillus subtilis
  source 1..3582: mol_type = genomic DNA
ttgacaggtcaactagttcagtatggacgacaccgccagcgcagaagctatgctcgcattagcgaagtgttagaattaccaaatctcattgaaattcaaacctcttcttatcagtggtttcttgatgagggtcttagagagatgtttcaagacatatcaccaattgaggatttcactggtaacctctctcttgagttcattgattatagtttaggtgagcctaaatatcctgtagaggaatcaaaagaacgtgatgtgacttactcagctccgctaagagtgaaggttcgtttaattaacaaagaaactggagaggtaaaagaccaagatgtcttcatgggtgatttccctattatgacagatacaggtacttttatcattaacggtgcggaacgtgttatcgtttcccagcttgttcggtctccaagtgtatatttcagtggtaaagtagacaaaaacggtaaaaaaggttttaccgcaactgtcattccaaaccgtggcgcatggttagaatacgaaactgatgcgaaagatgttgtttatgtccgcattgatcgcacacgtaagttgccggttacggttcttttgcgtgctctcggcttcggctccgatcaagagattcttgatctcataggagaaaacgaatacctgcgaaatacgcttgataaagataacacagaaaacagcgacaaagcgttgctggaaatttacgagcgtctccgtcctggagagccgcctacagtagaaaatgcgaaaagcttgcttgattctcgtttctttgatccgaaacgatacgatcttgccaatgtaggacgctataaaattaataaaaaacttcatattaagaatcgcctcttcaatcagagacttgctgaaacgcttgttgatcctgaaacaggagaaatccttgctgaaaaaggccagattcttgatagaagaacgcttgataaagtactgccatacttagaaaacggaatcggttttagaaagctgtatccgaatggcggcgttgttgaagatgaagtgactcttcaatcaattaaaatctttgctccgactgatcaagaaggagaacaggttatcaatgtaatcggcaatgcttacatcgaagaagagattaaaaacatcacgcctgctgatattatttcttcaatcagctacttcttcaacctgctgcacggagtaggcgacacagatgatatcgatcatcttggaaaccgccgtttacgttctgtaggcgagcttctccagaaccaattccgtatcggtttaagccgtatggagcgtgtggttcgtgagagaatgtcaattcaagatacgaatacaattacgcctcagcagctgatcaatattcgtcctgttattgcgtccattaaagagttctttggaagctcacagctttctcaattcatggatcagacgaacccgcttgctgaattaacgcacaagcgtcgtctgtcagcattaggaccgggcggattgacacgtgagcgtgccggaatggaagtgcgtgacgttcactactcccactatggccgtatgtgtccgattgaaacgcctgagggcccgaacatcggtttgatcaactcactatcatcttatgcaaaagtaaaccgttttggctttattgaaacgccatatcgccgcgttgaccctgaaacagggaaggtaacgggcagaatcgattacttaactgctgatgaagaggataactatgttgtcgctcaagcgaatgctcgtcttgatgacgaaggcgcctttattgatgacagcatcgtagctcgtttccgcggggagaacaccgttgtttccagaaatcgtgtagactacatggatgtatcgcctaagcaggttgtatctgctgcgacagcatgtatcccgttcttagaaaacgatgactccaaccgtgccctcatgggagcgaacatgcagcgtcaggctgtgcctttgatgcagccggaagcgccatttgttggaactggtatggaatacgtatcaggaaaagactctggtgccgctgttatttgtaaacaccctggtatcgttgaacgcgtagaagccaaaaacgtttgggttcgccgttatgaagaagtagacggtcaaaaagtaaaaggaaacctggataaatacagcctgctgaaatttgtccgctctaaccaaggtacgtgctacaaccagcgtccgatcgtaagtgtcggcgatgaagtggtaaaaggagaaatccttgctgacggtccttctatggagcttggtgaacttgcacttggccgtaacgtaatggtcggcttcatgacgtgggatggctacaactatgaggatgccatcatcatgagtgaacgcctagtgaaggatgatgtttatacatctatccacattgaagaatacgaatcagaagcacgtgatacgaaacttggacctgaagaaatcactcgcgatattccaaacgtcggtgaagatgcgcttcgcaatcttgatgaccgcggaatcatccgtattggggcagaagtaaaagacggagatcttcttgttggtaaagtaacgcctaaaggcgtaactgaactgactgccgaagaacgccttcttcacgccatctttggcgagaaagcccgcgaggttcgtgatacttctcttcgtgtgcctcatggcggcggcggaattatccatgacgttaaagtcttcaaccgtgaagacggagacgaacttcctccaggtgttaaccagttagtacgcgtatatatcgttcagaaacgtaagatttctgaaggggataaaatggccggtcgtcacggtaacaaaggtgttatctctaagattcttcctgaagaggatatgccttaccttcctgacggcacaccaattgatatcatgcttaacccgctgggcgtaccatcacgtatgaacatcgggcaggtattggaacttcacatgggtatggccgctcgttaccttggcattcacattgcatctcctgtatttgacggagcgcgagaagaggatgtctgggaaacacttgaagaagccggcatgtctcgtgacgccaaaacagtgctttacgacggacgtactggagagccgtttgataaccgtgtatctgtcggtatcatgtacatgatcaaactggctcacatggttgacgataaacttcatgcacgctctacaggcccttactcacttgttacgcagcagcctcttggcggtaaagcgcaatttggcggacagcgttttggtgagatggaggtttgggcacttgaagcttacggtgcggcttacactcttcaagaaattctgactgttaagtctgatgacgtggttggacgtgtgaaaacatacgaagccatcgttaaaggcgacaatgttcctgaaccaggtgttccggaatcattcaaagtattaatcaaagaacttcaaagcttaggtatggatgtcaaaatcctttctggtgatgaagaagaaatagaaatgagagatttagaagacgaagaagatgcgaaacaagctgacggcctggcattatcaggtgatgaagagccggaagaaacagcatctgcagacgttgaacgcgatgtagtaacaaaagaataa

SEQ ID NO: 5 - DNA, 1197 bp, Bacillus subtilis
  source 1..1197: mol_type = genomic DNA
gtgaaaaataaatggctgtcttttttttcgggtaaggtccagcttgaattgacgggaagagggattgagcggctccttaatgaatgcacaagacaggggattccggtctttcatgtcaaaaaaaagaaagaagccgtatcgttatatatacagcttcaggatgtacatgcctttcggcgggtgagaagtaaatttaaatgtaaagcccgatttatcaatcggaagggatttcccttcctgttgctgaaatcaaagctgaatatagggtttacgatcggttttgcgatttttttcatccttttgtttttgctgtccaatatggtgtggaaaattgatgtgacaggcgctaagcctgaaacagaacatcaaatgaggcagcatcttaatgaaatcggcgtcaaaaagggccgtctgcagtttttaatgatgtcgcccgaaaaaatacagaaatcattaaccaatggaatagacaatatcacttgggtcggagttgatctgaaggggacgaccattcacatgaaagttgtggagaaaaatgagcccgaaaaagaaaagtatgttagcccgcgcaatattgtcgccaaaaagaaagcaaccattacgagaatgtttgtgcaaaaaggacagcccatggccgccatacacgatcatgttgaaaaggggcagctgcttgtttcgggactgatcggcagcgaagaccatcagcaggaagttgcctcaaaagcagaaatttacggagaaacctggtatagatcagaagtgacagtcccgcttgaaacattatttaacgtctatacgggcaaagtaaggacaaagcacaagctttcttttggttctttggcaatcccgatctgggggatgacgtttaaaaaagaggaattgaagcatccaaaaacagaacaagaaaaacattcgcttcattttctcggatttaagctccctgtatcctatgtcaaagagcaaacgagagaaagtgaagaggctttgcgaaaatatacaaaagaagaagccgttcaagaaggcattaaattgggtaaacaggatgtagaggataaaataggcgaaaacggcgaggtgaaaagtgaaaaagttttgcaccagactgttgagaatggtaaagtaaagttgattattctctaccaagttatagaagatatcgttcaaaccacacctattgtcagggagactgaagaatga

SEQ ID NO: 6 - DNA, 585 bp, Bacillus subtilis
  source 1..585: mol_type = genomic DNA
atggggacttcacaagaacaggaaagcactgtacagatcaattcacaagaacaggaaaacaccgaacaaattagttatccgagtgttgaaactcttctatctactgtcaccagagaatacgacacagaagctaatagaaaaagagatattgaaactagagctggtgtcctcattgccctgttaggtgctttaataggattttatacatcagctttggatttttcattttttaaaaaagcaaatagttcaatagaaattctctgttttgtaatagtaagtgtattgtatatattccccgcaattatgcaattaattgcttttaaacatttgattaatgtcttaaaaacttacgaatatgacactcttggtttaggcggattcgacaaagaacacgttgcacaaaaacctaaagagaatcttcaatttaatttgacaaaacaatacaaaaaaataattgttgtcaatcgtaaagcaaatgatactaaagttgaacttttcaaaaaaggaattaaagagatttacatatctataattggcatagtagttgtatattttatgaaacaaatattacttctaattgtttaa

SEQ ID NO: 7 - DNA, 1457 bp, Bacillus subtilis
  source 1..1457: mol_type = genomic DNA
gttagcggcggacgggtgagtaacacgtgggtaacctgcctgtaagactgggataactccgggaaaccggggctaataccggatggttgtttgaaccgcatggttcaaacataaaaggtggcttcggctaccacttacagatggacccgcggcgcattagctagttggtgaggtaacggctcaccaaggcaacgatgcgtagccgacctgagagggtgatcggccacactgggactgagacacggcccagactcctacgggaggcagcagtagggaatcttccgcaatggacgaaagtctgacggagcaacgccgcgtgagtgatgaaggttttcggatcgtaaagctctgttgttagggaagaacaagtaccgttcgaatagggcggtaccttgacggtacctaaccagaaagccacggctaactacgtgccagcagccgcggtaatacgtaggtggcaagcgttgtccggaattattgggcgtaaagggctcgcaggcggtttcttaagtctgatgtgaaagcccccggctcaaccggggagggtcattggaaactggggaacttgagtgcagaagaggagagtggaattccacgtgtagcggtgaaatgcgtagagatgtggaggaacaccagtggcgaaggcgactctctggtctgtaactgacgctgaggagcgaaagcgtggggagcgaacaggattagataccctggtagtccacgccgtaaacgatgagtgctaagtgttagggggtttccgccccttagtgctgcagctaacgcattaagcactccgcctggggagtacggtcgcaagactgaaactcaaaggaattgacgggggcccgcacaagcggtggagcatgtggtttaattcgaagcaacgcgaagaaccttaccaggtcttgacatcctctgacaatcctagagataggacgtccccttcgggggcagagtgacaggtggtgcatggttgtcgtcagctcgtgtcgtgagatgttgggttaagtcccgcaacgagcgcaacccttgatcttagttgccagcattcagttgggcactctaaggtgactgccggtgacaaaccggaggaaggtggggatgacgtcaaatcatcatgccccttatgacctgggctacacacgtgctacaatggacagaacaaagggcagcgaaaccgcgaggttaagccaatcccacaaatctgttctcagttcggatcgcagtctgcaactcgactgcgtgaagctggaatcgctagtaatcgcggatcagcatgccgcggtgaatacgttcccgggccttgtacacaccgcccgtcacaccacgagagtttgtaacacccgaagtcggtgaggtaaccttttaggagccagccgccgaaggtgggacagatgattggggtgaagtcgtaacaaggtagccgtatcggaaggtgcggctggatcacctccttt

SEQ ID NO: 8 - DNA, 1632 bp, Bacillus subtilis
  source 1..1632: mol_type = genomic DNA
atggcaaaagatattaagtttagtgaagaagctcgccgcgcaatgcttcgcggtgtcgatgcacttgctgatgctgttaaagtaactttaggaccaaaaggacgcaacgtggttctagagaaaaaattcggttctccgttaatcacaaatgacggtgtaacaatcgctaaagaaatcgagctagaagatgcgtttgaaaacatgggtgctaagcttgttgctgaagtagccagcaaaacaaacgacgttgccggtgacggtacaacaactgcaacagttcttgcgcaagcaatgatccgtgaaggccttaaaaacgtaacagcaggcgctaaccctgtaggcgtgcgtaaagggatggaacaagctgtagcggttgcgatcgaaaacttaaaaaaaatttctaagccaatcgaaggcaaagagtctatcgctcaggttgctgcgatctctgctgctgatgaggaagtcggaagccttatcgctgaagcaatggagcgcgtaggaaacgacggcgttatcacaatcgaagagtctaaaggcttcacaactgagcttgaagttgttgaaggtatgcaattcgaccgcggatatgcgtctccttacatggtaactgactctgataagatggaagcggttcttgacaatccttacatcttaatcacagacaaaaaaatcacaaacattcaagaaatccttcctgtgcttgagcaggttgttcagcaaggcaaaccattgcttctgatcgctgaggatgttgaaggcgaagcacttgctacacttgttgtgaacaaacttcgcggcacattcaacgcagtggctgttaaagctcctggcttcggtgatcgccgtaaagcaatgcttgaagacatcgctgtccttactggcggagaagtcatcacagaagatcttggccttgacctgaaatctactcaaatcgctcaattgggacgcgcttctaaagttgtcgttactaaagaaaacacaacaatcgttgaaggcgctggcgaaacagacaaaatttctgcccgtgtgactcaaatccgcgctcaagtggaagaaacaacttctgaattcgacagagaaaaattacaagagcgtcttgcgaaacttgctggcggcgtagctgtcatcaaagtcggcgctgcgactgaaactgagctgaaagagcgtaaacttcgcatcgaagacgccttgaactcaactcgcgcagctgttgaagaaggcatcgtatccggtggtggtacagcgcttgtaaacgtatataataaagtcgctgcagttgaagctgaaggcgatgctcaaacaggtatcaacatcgtgcttcgcgcgcttgaagagccaatccgtcaaatcgcacacaatgctggtcttgaaggatctgtcatcgttgaacgcctcaaaaacgaagaaatcggcgtaggcttcaacgctgcaactggcgaatgggtaaacatgatcgaaaaaggtatcgttgacccaacgaaagttacacgctcagctcttcaaaacgctgcgtctgtagctgcaatgttcttaacaactgaagccgttgtcgctgacaagccagaagaaaacgctggcggcggaatgcctgacatgggcggcatgggcggtatgggtggaatgatgtaa

SEQ ID NO: 9 - DNA, 1917 bp, Bacillus subtilis
  source 1..1917: mol_type = genomic DNA
atggaacagcagcaaaacagttatgatgaaaatcagatacaggtactagaaggattggaagctgttcgtaaaagaccggggatgtatatcggttcgacaaacagcaaaggccttcaccacttggtatgggaaattgtcgacaatagtattgacgaagccctcgccggttattgtacggatatcaatatccaaatcgaaaaagacaacagtatcacggttgtagataatggccgcggtattccagtcggtattcatgaaaaaatgggccgtcctgcggtagaagtcattatgacggtgcttcatgccggaggaaaatttgacggaagcggctataaagtatccggaggattacacggtgtaggtgcgtcggtcgtaaacgcactatcaacagagcttgatgtgacggttcaccgtgacggtaaaattcaccgccaaacctataaacgcggagttccggttacagaccttgaaatcattggcgaaacggatcatacaggaacgacgacacattttgtcccggaccctgaaattttctcagaaacaaccgagtatgattacgatctgcttgccaaccgcgtgcgtgaattagcctttttaacaaagggcgtaaacatcacgattgaagataaacgtgaaggacaagagcgcaaaaatgaataccattacgaaggcggaattaaaagttatgtagagtatttaaaccgctctaaagaggttgtccatgaagagccgatttacattgaaggcgaaaaggacggcattacggttgaagtggctttgcaatacaatgacagctacacaagcaacatttactcgtttacaaacaacattaacacgtacgaaggcggtacccatgaagctggcttcaaaacgggcctgactcgtgttatcaacgattacgccagaaaaaaagggcttattaaagaaaatgatccaaacctaagcggagatgacgtaagggaagggctgacagcgattatttcaatcaaacaccctgatccgcagtttgagggccaaacgaaaacaaagctgggcaactcagaagcacggacaatcaccgatacgttattttctacagcgatggaaacatttatgctggaaaatccagatgcagccaaaaaaattgttgataaaggcttaatggcggcaagagcaagaatggctgcgaaaaaagcgcgtgaactaacacgccgtaagagtgctttggaaatttcaaacttgcccggtaagttagcggactgctcttcaaaagatccgagcatttccgagttatatatcgtagagggtgactctgccggaggatctgctaaacaaggacgcgacagacatttccaagccattttgccgcttagaggtaaaatcctaaacgttgaaaaggccagactggataaaatcctttctaacaacgaagttcgctctatgatcacagcgctcggcacaggcatcggggaagacttcaaccttgagaaagcccgttaccacaaagttgtcattatgacagatgccgatgttgacggcgcgcacatcagaacacttctgttaacgttcttttacagatatatgcgccaaattatcgaaaatggctacgtgtacattgcgcagccgccgctctacaaggttcaacaggggaaacgcgttgaatatgcgtacaatgacaaggagcttgaagagctgttaaaaactcttcctcaaacgcctaagcctggactgcagcgttacaaaggtcttggtgaaatgaatgccacccagctatgggagacaaccatggatcctagttccagaacacttcttcaggtaactcttgaagatgcaatggatgcggacgagacttttgaaatgcttatgggcgacaaggtagaaccgcgccgaaacttcatagaagcgaatgcgagatacgttaaaaatcttgacatctaa

SEQ ID NO: 10 - DNA, 3582 bp, Bacillus subtilis
  source 1..3582: mol_type = genomic DNA
ttgacaggtcaactagttcagtatggacgacaccgccagcgcagaagctatgctcgcattagcgaagtgttagaattaccaaatctcattgaaattcaaacctcttcttatcagtggtttcttgatgagggtcttagagagatgtttcaagacatatcaccaattgaggatttcactggtaacctctctcttgagttcattgattatagtttaggtgagcctaaatatcctgtagaggaatcaaaagaacgtgatgtgacttactcagctccgctaagagtgaaggttcgtttaattaacaaagaaactggagaggtaaaagaccaagatgtcttcatgggtgatttccctattatgacagatacaggtacttttatcattaacggtgcagaacgcgttatcgtttcccagcttgttcggtctccaagtgtatatttcagtggtaaagtagacaaaaacggtaaaaaaggttttaccgcaactgtcattccaaaccgtggcgcatggttagaatacgaaactgatgcgaaagatgttgtttatgtccgcattgatcgcacacgtaagttgccggttacggttcttttgcgtgctctcggcttcggctccgatcaagagattcttgatctcataggagaaaacgaatacctgcgaaatacgcttgataaagataacacagaaaacagcgacaaagcgttgctggaaatttacgagcgtctccgtcctggagagccgcctacagtagaaaatgcgaaaagcttgcttgattctcgtttctttgatccgaaacgatacgatcttgccaatgtaggacgctataaaattaataaaaaacttcatattaagaatcgcctcttcaatcagagacttgctgaaacgcttgttgatcctgaaacaggagaaatccttgctgaaaaaggccagattcttgatagaagaacgcttgataaagtactgccatacttagaaaacggaatcggttttagaaagctgtatccgaatggcggcgttgttgaagatgaagtgactcttcaatcaattaaaatctttgctccgactgatcaagaaggagaacaggttatcaatgtaatcggcaatgcttacatcgaagaagagattaaaaacatcacgcctgctgatattatttcttcaatcagctacttcttcaacctgctgcacggagtaggcgacacagatgatatcgatcatcttggaaaccgccgtttacgttctgtaggcgagcttctccagaaccaattccgtatcggtttaagccgtatggagcgtgtggttcgtgagagaatgtcaattcaagatacgaatacaattacgcctcagcagctgatcaatattcgtcctgttattgcatccattaaagagttctttggaagctcacagctttctcaattcatggatcagacgaacccgcttgctgaattaacgcacaagcgtcgtctgtcagcattaggaccgggcggattgacacgtgagcgtgccggaatggaagtgcgtgacgttcactactcccactatggccgtatgtgtccgattgaaacgcctgagggcccgaacatcggtttgatcaactcactatcatcttatgcaaaagtaaaccgttttggctttattgaaacgccatatcgccgcgttgaccctgaaacagggaaggtaacgggcagaatcgattacttaactgctgatgaagaggataactatgttgtcgctcaagcgaatgctcgtcttgatgacgaaggcgcctttattgatgacagcatcgtagctcgtttccgcggggagaacactgttgtttccagaaaccgtgtagactacatggatgtatcgcctaagcaggttgtatctgctgcgacagcatgtatcccgttcttagaaaacgatgactccaaccgtgccctcatgggagcgaacatgcagcgtcaggctgtgcctttgatgcagccggaagcgccatttgttggaactggtatggaatacgtatcaggaaaagactctggtgccgctgttatttgtaaacaccctggtatcgttgaacgcgtagaagcgaaaaacgtttgggttcgccgttatgaagaagtagacggtcaaaaagtaaaaggaaacctggataaatacagcctgctgaaatttgtccgctctaaccaaggtacgtgctacaaccagcgtccgatcgtaagtgtcggcgatgaagtggtaaaaggagaaatccttgctgacggtccttctatggagcttggtgaacttgcacttggccgtaacgtaatggtcggcttcatgacgtgggatggctacaactatgaggatgccatcatcatgagtgaacgcctagtgaaggatgatgtttatacatctatccacattgaagaatacgaatcagaagcacgtgatacgaaacttggacctgaagaaatcactcgcgatattccaaacgtcggtgaagatgcgcttcgcaatcttgatgaccgcggaatcatccgtattggggcagaagtaaaagacggagatcttcttgttggtaaagtaacgcctaaaggcgtaactgaactgactgccgaagaacgccttcttcacgccatctttggcgagaaagcccgcgaggttcgtgatacttctcttcgtgtgcctcatggcggcggcggaattatccatgacgttaaagtcttcaaccgtgaagacggagacgaacttcctccaggtgttaaccagttagtacgcgtatatatcgttcagaaacgtaagatttctgaaggggataaaatggccggtcgtcacggtaacaaaggtgttatctctaagattcttcctgaagaggatatgccttaccttcctgacggcacaccaattgatatcatgcttaacccgctgggcgtaccatcacgtatgaacatcgggcaggtattggaacttcacatgggtatggccgctcgttaccttggcattcacattgcatctcctgtatttgacggagcgcgagaagaggatgtctgggaaacacttgaagaagccggcatgtctcgtgacgccaaaacagtgctttacgacggacgtactggagagccgtttgataaccgtgtatctgtcggtatcatgtacatgatcaaactggctcacatggttgacgataaacttcatgcacgctctacaggcccttactcacttgttacgcagcagcctcttggcggtaaagcgcaatttggcggacagcgttttggtgagatggaggtttgggcacttgaagcttacggtgcggcttacactcttcaagaaattctgactgttaagtctgatgacgtggttggacgtgtgaaaacatacgaagccatcgttaaaggcgacaatgttcctgaaccaggtgttccggaatcattcaaagtattaatcaaagaacttcaaagcttaggtatggatgtcaaaatcctttctggtgatgaagaagaaatagaaatgagagatttagaagacgaagaagatgcgaaacaagctgacggcctggcattatcaggtgatgaagagccggaagaaacagcatctgcagacgttgaacgcgatgtagtaacaaaagaataa

SEQ ID NO: 11 - DNA, 1197 bp, Bacillus subtilis
  source 1..1197: mol_type = genomic DNA
gtgaaaaataaatggctgtcttttttttcgggtaaggtccagcttgaattgacgggaagagggattgagcggctccttaatgaatgcacaagacaggggattccggtctttcatgtcaaaaaaaagaaagaagccgtatcgttatatatacagcttcaggatgtacatgcctttcggcgggtgagaagtaaatttaaatgtaaagcccgatttatcaatcggaagggatttcccttcctgttgctgaaatcaaagctgaatatagggtttacgatcggttttgcgatttttttcatccttttgtttttgctgtccaatatggtgtggaaaattgatgtgacaggcgctaagcctgaaacagaacatcaaatgaggcagcatcttaatgaaatcggcgtcaaaaagggccgtctgcagtttttaatgatgtcgcccgaaaaaatacagaaatcattaaccaatggaatagacaatattacttgggtcggagttgatctgaaggggacgaccattcatatgaaagttgtggagaaaaatgagcccgaaaaagaaaaatatgttagcccgcgcaatattgtcgccaaaaagaaagcaaccattacgagaatgtttgtgcaaaaaggacagcccatggccgccatacacgatcatgttgaaaagggacagctgcttgtttcgggactgatcggcagcgaagaccatcagcaggaagtcgcctcaaaagcagaaatttacggagaaacctggtatagatcagaagtgacagtcccgcttgaaacattatttaacgtctatacgggcaaagtaaggacaaagcacaagctttcttttggttctttggcaatcccgatctgggggatgacgtttaaaaaagaggaattgaagcatccaaaaacagaacaagaaaagcattcgcttcattttctcggatttaagctccctgtatcctatgtcaaagagcaaacgagagaaagtgaagaggctttgcgaaaatatacaaaagaagaagcagttcaagaaggcattaaattgggtaaacaggatgtagaggataaaataggcgaaaacggcgaggtgaaaagtgaaaaagttttgcaccagactgttgagaatggtaaagtaaagttgattattctctaccaagttatagaagatatcgttcaaaccacacctattgtcagggagactgaagaatga

SEQ ID NO: 12 - DNA, 1457 bp, Bacillus subtilis; identical to SEQ ID NO: 7
  source 1..1457: mol_type = genomic DNA

SEQ ID NO: 13 - DNA, 1635 bp, Bacillus subtilis
  source 1..1635: mol_type = genomic DNA
atggcaaaagaaattaagtttagtgaagaagctcgccgcgcaatgcttcgcggtgtcgatgcacttgctgatgctgttaaagtaactttaggaccaaaaggacgcaacgtggttctagagaaaaaattcggttctccgttaatcacaaatgacggtgtaacaatcgctaaagaaatcgagctagaagacgcgtttgaaaacatgggtgctaagcttgttgctgaagtagccagcaaaacaaacgacgttgccggtgacggtacaacaactgcaacagttcttgcgcaagcaatgatccgtgaaggccttaaaaacgtaacagcaggcgctaaccctgtaggcgtgcgtaaagggatggaacaagctgtagcggttgcgatcgaaaacttaaaagaaatttctaagccaatcgaaggcaaagagtctatcgctcaggttgctgcgatctctgctgctgatgaggaagtcggaagccttatcgctgaagcaatggagcgcgtaggaaacgacggcgttatcacaatcgaagagtctaaaggcttcacaactgagcttgaagttgttgaaggtatgcaattcgaccgcggatatgcgtctccttacatggtaactgactctgataagatggaagcggttcttgacaatccttacatcttaatcacagacaaaaaaatcacaaacattcaagaaatccttcctgtgcttgagcaggttgttcagcaaggcaaaccattgcttctgatcgctgaggatgttgaaggcgaagcacttgctacacttgttgtgaacaaacttcgcggcacattcaacgcagtggctgttaaagctcctggtttcggtgatcgccgtaaagcaatgcttgaagacatcgctgtccttactggcggagaagtcatcacagaagatcttggccttgacctgaaatctactcaaatcgctcaattgggacgcgcttctaaagttgtcgttactaaagaaaacacaacaatcgttgaaggcgctggcgaaacagacaaaatttctgcccgtgtgactcaaatccgcgctcaagtggaagaaacaacttctgaattcgacagagaaaaattacaagagcgtcttgctaaacttgctggcggcgtagctgtcatcaaagtcggcgctgcgactgaaactgagctgaaagagcgtaaacttcgcatcgaagacgccttgaactcaactcgcgcagctgttgaagaaggcatcgtatccggtggtggtacagcgcttgtaaacgtatataacaaagtcgctgcagttgaagctgaaggcgatgctcaaacaggtatcaacatcgtgcttcgcgcgcttgaagagccaatccgtcaaatcgcacacaacgctggccttgaaggatctgtcatcgttgagcgcctcaaaaacgaagaaatcggcgtaggcttcaacgctgcaactggcgaatgggtaaacatgatcgaaaaaggtatcgttgacccaacaaaagttacacgctcagctcttcaaaacgctgcgtctgtagctgcaatgttcttaacaacagaagctgttgtcgctgacaagccagaagaaaacggtggcggcgcaggaatgcctgatatgggcggcatgggcggtatgggtggaatgatgtaa

SEQ ID NO: 14 - DNA, 1917 bp, Bacillus subtilis
  source 1..1917: mol_type = genomic DNA
atggaacagcagcaaaacagttatgatgaaaatcagatacaggtactagaaggattggaagctgttcgtaaaagaccggggatgtatatcggttcgacaaacagcaaaggccttcaccacttggtatgggaaattgtcgacaatagtattgacgaagccctcgccggttattgtacggatatcaatatccaaatcgaaaaagacaacagtatcacggttgtagataatggccgcggtattccagtcggtattcatgaaaaaatgggccgtcctgcggtagaagtcattatgacggtgcttcatgccggaggaaaatttgacggaagcggctataaagtatccggaggattacacggtgtaggtgcgtcggtcgtaaacgcactatcaacagagcttgatgtgacggttcaccgtgacggtaaaattcaccgccaaacctataaacgcggagttccggttacagaccttgaaatcattggcgaaacggatcatacaggaacgacgacacattttgtcccggaccctgaaattttctcagaaacaaccgagtatgattacgatctgcttgccaaccgcgtgcgtgaattagcctttttaacaaagggcgtaaacatcacgattgaagataaacgtgaaggacaagagcgcaaaaatgaataccattacgaaggcggaattaaaagttatgtagagtatttaaaccgctctaaagaggttgtccatgaagagccgatttacattgaaggcgaaaaggacggcattacggttgaagtggctttgcaatacaatgacagctacacaagcaacatttactcgtttacaaacaacattaacacgtacgaaggcggtacccatgaagctggcttcaaaacgggcctgactcgtgttatcaacgattacgccagaaaaaaagggcttattaaagaaaatgatccaaacctaagcggagatgacgtaagggaagggctgacagcgattatttcaatcaaacaccctgatccgcagtttgagggccaaacaaaaacaaagctgggcaactcagaagcacggacgatcaccgatacgttattttctacggcgatggaaacatttatgctggaaaatccagatgcagccaaaaaaattgtcgataaaggtttaatggcggcaagagcaagaatggctgcgaaaaaagcgcgtgaactaacacgccgtaagagtgctttggaaatttcaaacctgcccggtaagttagcggactgctcttcaaaagatccgagcatctccgagttatatatcgtagagggtgactctgccggaggatctgctaaacaaggacgcgacagacatttccaagccattttgccgcttagaggtaaaatcctaaacgttgaaaaggccagactggataaaatcctttctaacaacgaagttcgctctatgatcacagcgctcggcacaggtatcggagaagacttcaaccttgagaaagcccgttaccacaaagttgtcattatgacagatgccgatgttgacggcgcgcacatcagaacactgctgttaacgttcttttacagatatatgcgccaaattatcgaaaatggctacgtgtacattgcgcagccgccgctctacaaggttcaacaggggaaacgcgttgaatatgcatacaatgacaaggagcttgaagagctgttaaaaactcttcctcaaacgcctaagcctggactgcagcgttacaaaggtcttggtgaaatgaatgccacccagctatgggagacaaccatggatcctagctccagaacacttcttcaggtaactcttgaagatgcaatggatgcggatgagacttttgaaatgcttatgggcgacaaggtagaaccgcgccgaaacttcatagaagcgaatgcgagatacgttaaaaatcttgacatctaa

SEQ ID NO: 15 - DNA, 3582 bp, Bacillus subtilis; identical to SEQ ID NO: 4
  source 1..3582: mol_type = genomic DNA

SEQ ID NO: 16 - DNA, 1197 bp, Bacillus subtilis
  source 1..1197: mol_type = genomic DNA
gtgaaaaataaatggctgtcttttttttcgggtaaggtccagcttgaattgacgggaagagggattgagcggctccttaatgaatgcacaagacaggggattccggtctttcatgtcaaaaaaaagaaagaagccgtatcgttatatatacagcttcaggatgtacatgcctttcggcgggtaagaagtaaatttaaatgtaaagcccgatttatcaatcggaagggatttcccttcctgttgctgaaatcaaagctgaatatagggtttacgatcggttttgcgatttttttcattcttttgtttttgctgtccaatatggtgtggaaaattgatgtgacaggcgctaagcctgaaacagaacatcaaatgaggcagcatcttaatgaaatcggcgtcaaaaagggccgtctgcagtttttaatgatgtcgcccgaaaaaatacagaaatcattaaccaatggaatagacaatatcacttgggtcggagttgatctgaaggggacgaccattcatatgaaagttgtggagaaaaatgagcccgaaaaagaaaaatatgttagcccgcgcaatattgtcgccaaaaagaaagcaaccattacgagaatgtttgtgcaaaaaggacagcccatggccgccatacacgatcatgttgaaaagggacagctgcttgtttcgggactgatcggcagcgaagaccatcagcaggaagtcgcctcaaaagcagaaatttatggagaaacctggtatagatcagaagtgacagtcccgcttgaaacattatttaacgtctatacgggcaaagtaaggacaaagcacaagctttcttttggttctttggcaatcccgatctgggggatgacgtttaaaaaagaggaattgaagcatccaaaaacagaacaagaaaagcattcgcttcattttctcggatttaagctccctgtatcctatgtcaaagagcaaacgagagaaagtgaagaggctttgcgaaaatatacaaaagaagaagcagttcaagaaggcattaaattgggtaaacaggatgtagaggataaaataggcgaaaacggcgaggtgaaaagtgaaaaagttttgcaccagactgttgagaatggtaaagtaaagttgattattctctaccaagttatagaagatatcgttcaaaccacacctattgtcagggagactgaagaatga

SEQ ID NO: 17 - DNA, 2565 bp, Bacillus subtilis
  source 1..2565: mol_type = genomic DNA
gtggcattcagattaattaaagattatgacacaacccgaaacgcaagatatatcgcgcagcaaagagcagatacagaaactatagaagatgggttgaacagtcttgatgatgcgattaaaacgcataaaacgtctcaaacggctcatacttccgatcaaattacccatcaaggtttttctctccgaacatatgttgaaagcctttataaccgtatgcgtaatttgattcttaatgctgacggaacaaacgtaaaagaggtcgtcgatgcccgtgttgatactgacggcaatattgcgcccttattaaaagaacggcttgaccgggagtaccttaagcttctacagaagatcaaacggacggttaacgttgatgacttcggagcagatccgactggcgttaacgatagtacagaagcgtttcagagggcgatcggtgccggtaaagtccgtattaatttatcggcgggcacgtatatcgtaaagggcgttaaactgccatcgtggacttatatggtaggacaaggaatcggagttacaacgttgaagctccacgaagacacgccggctagcgaatgggtggtcactaacgcggaccatgccggaggcaaccgaaatattaccgtcgaaggtatgacgctagattggaatccggaacgtcaaggtggcgtaggagcaacgggtgggctgcactcgagcggtctgacattcgcgcaagtaaagttcggtatcgtacgcgaagtggagagtgttaagccgggccttcatagtttcgatgcctcagcgccaacttacgatattagagcaacggactatacgaagcagggttgtcggtatatctggttcgatcgctgcgtcggctctggatacggggatgacgggatttccacgcattacagcgagtacatttttattacgaattgcattatgacgaacccgagaggaactgctcacgctgcgggaagagctaattccaacggtattgaggtggatgacggatctaaaaacgtatgggtaattgactgttataccgaaggcaatgtaaggggagtcgaagtgaaagcacacgcagcttggccggcaccttcaaatgttcatattcgcggacacgaatcctatcgtgatgtacgtgcttatgatcttcgccatattggccatcatttagaagccgacccttggagtgaatcagcgcgcgacataacgatcgttgattgtactgcccgtgagcctatatataacgatctatacgagggtatggttccaaaggctctcgtaatatcggcatatcagcgcgtcatggtttccaatttccgtgcgataggcgacccgacttacgattataaaggagcgccaattatcgccttccagtataaaagccggaagattaacgttgatggacttcagattagcggattcgccaaagctggatcagacatccatatttacggaggcggacagcggacggatgatgttcatatttcgaattttacgatccacgattcggcaccagtcggaatcagtataggaggcggagtttacttcgttactttgatgaacgggattgcgcacacgcgcggagggacttccggtatcacctcgccgaacaaccaggcgaatatcattgcggttcgtgctgtcggatacacggatgcagcggtattaggcggacaaaaatataaagtcgtcccgaataacatcaaaggcggattccgtgcggcttcttccacaggggccactttgactgattccagcgccatcatcgcgaacaccggatcagctatcgcaaagggtgagcgcaactttatcgccggtaatgcgggtggagcatctaccgaaggttcgcggaatggagttatgttctcgtacgattcgcatacaacaggcgacggcggttcgtccggtgttatgttttcgcgtgcaacgaagaacagcaaatcgtattcacttgcgatggggcatggcacaggcagcgcatcagaagcgaacaagaaaatcgaactaagcgcagaatacggaaccgtaagagcaaccggcgcagtcgaaagcgtatcaaaccttcgggatttcgcggagtactttgaatcgatagacggtaagaaaatcgatgcctcgtatctagttgcgttagaaggcgacaagatacgaaaagctgataaaggcgataagatcctgggcgttgtttctaaaactgcgggcttggtactcggtggagcagcgttctattggaatgaccgttacctacacgacgagttcggcggacttatctatcatgaaatcgttgaggatggtcgtacggtcaccgtacctgtcgagaatccggactacgatccaaccgtagaatatacacctcgcgaagaaagagacgaatggcacgtagtcggattgatcgggcaagtttatgtgcgtatcgacgaaaccgtcgcggtaggagacagcgtgactgcggtcggtggtgtcgcaacaaaagcggaatcaaacggatacggaacggtcatgaaaataaaaacgccttataacgcagaaaaaggctatggcgtagcgcagatgatcgtcacgccgcagcattaa

SEQ ID NO: 18 - DNA, 1456 bp, Bacillus pumilus
  source 1..1456: mol_type = genomic DNA
gttagcggcggacgggtgagtaacacgtgggtaacctgcctgtaagactgggataactccgggaaaccggagctaataccggatagttccttgaaccgcatggttcaaggatgaaagacggtttcggctgtcacttacagatggacccgcggcgcattagctagttggtggggtaatggctcaccaaggcgacgatgcgtagccgacctgagagggtgatcggccacactgggactgagacacggcccagactcctacgggaggcagcagtagggaatcttccgcaatggacgaaagtctgacggagcaacgccgcgtgagtgatgaaggttttcggatcgtaaagctctgttgttagggaagaacaagtgcgagagtaactgctcgcaccttgacggtacctaaccagaaagccacggctaactacgtgccagcagccgcggtaatacgtaggtggcaagcgttgtccggaattattgggcgtaaagggctcgcaggcggtttcttaagtctgatgtgaaagcccccggctcaaccggggagggtcattggaaactgggaaacttgagtgcagaagaggagagtggaattccacgtgtagcggtgaaatgcgtagagatgtggaggaacaccagtggcgaaggcgactctctggtctgtaactgacgctgaggagcgaaagcgtggggagcgaacaggattagataccctggtagtccacgccgtaaacgatgagtgctaagtgttagggggtttccgccccttagtgctgcagctaacgcattaagcactccgcctggggagtacggtcgcaagactgaaactcaaaggaattgacgggggcccgcacaagcggtggagcatgtggtttaattcgaagcaacgcgaagaaccttaccaggtcttgacatcctctgacaaccctagagatagggctttcccttcggggacagagtgacaggtggtgcatggttgtcgtcagctcgtgtcgtgagatgttgggttaagtcccgcaacgagcgcaacccttgatcttagttgccagcatttagttgggcactctaaggtgactgccggtgacaaaccggaggaaggtggggatgacgtcaaatcatcatgccccttatgacctgggctacacacgtgctacaatggacagaacaaagggctgcgagaccgcaaggtttagccaatcccataaatctgttctcagttcggatcgcagtctgcaactcgactgcgtgaagctggaatcgctagtaatcgcggatcagcatgccgcggtgaatacgttcccgggccttgtacacaccgcccgtcacaccacgagagtttgtaacacccgaagtcggtgaggtaacctttatggagccagccgccgaaggtgggacagatgattggggtgaagtcgtaacaaggtagccgtatcggaaggtgcggctggatcacctccttt

SEQ ID NO: 19 - DNA, 1635 bp, Bacillus pumilus
  source 1..1635: mol_type = genomic DNA
atggcaaaagatattaagttcagtgaagaagcacgtcgcgcgatgttacgtggtgtagatgcacttgcagatgctgtaaaagtaactttaggacctaaaggacgtaacgtggttcttgagaaaaaattcggttctccacttatcacaaatgatggtgtgacgatcgcaaaagaaatcgaattagaagatgcatttgaaaacatgggtgcaaaacttgtggctgaagttgcaagcaaaacaaacgacgtagctggtgacggtacaacgactgcaacagttctagctcaagcgatgatccgtgaaggtcttaaaaacgtaacagctggtgcaaaccctgttggtgtacgtaaagggatcgaagaagcagtgaaagtagctcttgaaggcttgcacgagatttctaaaccaatcgaaggcaaagaatcaattgctcaagttgcgtctatttctgcagcagatgaagaagtgggaagccttatcgctgaagcaatggagcgtgtaggtaacgacggcgtcatcactatcgaagaatctaaaggtttcacaactgagctagaagtggttgaaggaatgcagtttgaccgcggatatgcttcaccatacatggtgacggattctgataagatggaagcggttcttgaaaatccttacatcttaatcactgataaaaaaatcacaaacattcaagaaatccttcctgtacttgagcaagttgtacaacaaggaaaaccattgttgatcattgcagaagatgtagaaggcgaagcacttgcaacacttgttgtaaacaaacttcgtggaacatttaacgcagtggcagtaaaagcacctggattcggtgatcgtcgtaaagcaatgcttgaagacatctctgttctaactggcggagagttaatcacagaagacctaggacttgacctgaaatcaactgaaatcggtcagcttggccgagcgtctaaagtcgttgtgacaaaagaaaacacaaccatcgtagaaggctcaggagattctgctcaaatcgcagcacgcgtgaaccaaatccgtgcgcaagttgaagaaacaacttctgaattcgataaagaaaaattacaagaacgtcttgctaaactagctggtggcgtcgctgtcatcaaagttggtgctgcaactgaaacagaactaaaagagcgtaaactacgcatcgaggatgcactcaactcaactcgtgcagcagttgaagaaggtatcgtatccggtggtggtacagcacttgtgaatgtatacaaaaaagtcgcttcaatcgaagcagatggtgacgttcaaacaggtgtgaacatcgttctacgttctcttgaagagccaatccgtcaaatcgctcacaacgcaggtcttgaaggatcagtcatcgttgagcgcttgaaaaacgaagaaattggcgtaggcttcaacgcagcaacaaacgaatgggtaaacatgatcgaaaaaggaatcgttgacccaacaaaagtaactcgttctgcacttcaaaacgcagcttctgttgcagcaatgcttctaacaactgaagcagtcgttgctgacaaaccagaagaaggcggctcaggcggcggaatgccggatatgggcggcatgggcggcatgggtggcatgatgtaa

SEQ ID NO: 20 - DNA, 1917 bp, Bacillus pumilus
  source 1..1917: mol_type = genomic DNA
atggaacagcaacataatagttatgatgaaaatcagatacaggtgcttgaaggactagaagctgttagaaaacgtccaggaatgtacattgggtcaaccagtgcaaaaggacttcaccatcttgtatgggaaattgtcgacaacagtattgatgaggctttagctggatattgcacagatattacggtgcaaattgaaaaggataatagcattacagtgaaagataatggccgcggaattcctgttgggattcatgagaaaatgggacgtcctgctgtagaggttattatgactgttcttcacgctggcggtaaatttgacggcagcggttataaagtatctggcggtctgcatggcgtaggggcatctgttgttaatgcgttatctacgaccttagacgtgaccgtatatcgtgatgggaaaattcattatcaacaattcaaacgcggtgttccagttggagatttagagatcattggtgaaacagatgttacagggacaaccactcattttgtgccagatacagaaatttttactgaaaccattgaatttgattacgacacacttgccaaccgtgtacgtgagttagctttcttaacaaaaggtgtcaacatcgttattgaagatttacgtgaggggaaagaacgacgaaatgaatactgctatgaaggcggtattaagagctatgtagaacatttaaatcgctcaaaagaagtcgttcatgaagaacccgtttacattgaaggtgaaaaagatggaatcacggttgaagtggcattacaatataacgattcctatacaagcaacatctattccttcgccaacaatatcaacacgtatgaaggcggaacacacgaagcaggctttaaaacagggctgacgcgtgtcatcaatgattatgctcgtaaaaatggcgtattcaaagatggagactcgaatttgagcggtgaagatgtgcgagaaggcttaacagccattatctccatcaagcatccaaatcctcaattcgaaggacaaacgaagacaaagcttgggaactcagaagcaagaaccattaccgactcccttttctctgaagcacttgagaaattcctcttagagaaccctgatgctgcaaagaaaattgtggagaaaggcgtgatggcagctcgtgcaagaatggctgccaaaaaggcacgtgagctgacaagacgtaaaagtgcactggaagtctccagcttaccggggaaactggcggactgttcttctaaagatccttccatctctgaactttatatcgtagagggagattctgcgggcggatctgctaagcaaggccgtgatcgtcacttccaagcgatcttaccgttaagagggaagatcttaaacgttgaaaaagcgcgactagataaaattctatcgaacaacgaagttcgttctatgattacagcgttaggaactggaatcggtgaagacttcactttagagaaagctcgctatcacaaagttgtgatcatgacggatgcggatgtcgatggtgcccatattcgcacgctgctcttaacgttcttctatcgctacatgcgtgaaatcattgaaaacggttatgtgtatattgcgcagccacctttatttaaagtgcagcaaggtaaacgtgttgagtatgtgtataacgataaacagctagatgagctgctaaagacattgcctcaaacaccaaaacctggacttcagcgctataaaggtcttggagaaatgaacgcaactcagctttgggaaacaacaatggatcctgatgcgagaacacttcttcaagtgacgcttgaggatgcgattgatgctgatgagacatttgaaatgttgatgggagataaagtagaaccgagacgaaactttatcgaagaaaatgcacaatacgtgaaaaatcttgatatttag

SEQ ID NO: 21 - DNA, 3582 bp, Bacillus pumilus
  source 1..3582: mol_type = genomic DNA
ttgacaggtcaactagttcagtatggacgacaccgccagcgcagaagctacgcacgcataagcgaagtgttagaattaccaaatctcattgaaattcaaacctcttcttatcagtggtttcttgatgagggtcttagagagatgtttcaagatatatccccaattgaggattttactggtaacctttctcttgaattcattgattacagcctaggggatcctaagtatcctgtagcagaatcaaaagaacgtgatgtaacttactctgctccactaagagtgaaagttcgtttaattaacaaagaaactggagaagtaaaagaccaagatgtgttcatgggtgatttcccaatcatgacagacacaggtacttttatcattaacggggcggaacgtgtaatcgtttctcagttagtacgttctccaagtgtatatttcagtggtaaagtagacaaaaacggtaaaaaaggttttactgcgactgtcattccaaaccgtggcgcatggttagaatacgaaactgatgcgaaggatgtagtctatgtacgcatcgatcgcacacgtaagttgccggttacggttcttttgcgtgctctcggcttcagctctgatcaagagattcttgacctcattggcgagaatgaatacttacgcaacacgctggaaaaagacaatacagagaatgctgataaagcacttctcgaaatctacgagcgcctccgtcctggagagccgccaactgttgaaaatgcgaaaagcctgctagactctcgcttcttcgatccgaagagatatgacctagcaaatgttggacgctacaagattaataaaaagcttcatattaaaaatagactgttcaatcaaaaattggctgaaacgttagttgaccctgaaacaggtgaaattctagcagaaaaaggtcaaattttagacagaagagttcttgataaagttcttccatacttagaaaacggcatcggatttagaaagctttatccaaatggtggcgtagtagaagatgaagtagaacttcaatctattaagatttatgcaccgtctgatcaagaaggcgagcaagtgatcaacgtgatcgggaatgcatacgtagaggaagctgtgaaaaacatcacgccttctgacatcattgcatcgatcagttacttcttcaaccttcttcatggtgtaggtgacacagatgatatcgatcaccttggtaaccgtcgcctgcgttctgtaggtgaacttctgcaaaaccaattccgtattggtttaagcagaatggagcgtgttgttcgtgaaagaatgtcgatccaagacacaaacacgatcacacctcagcaactgatcaacatccgtcctgtgatcgcttctatcaaagagttctttggtagctctcagctttctcagttcatggatcaaacaaacccgcttgctgaattgacgcacaaacgtcgtctgtcagcgcttgggcctggtggtttgacacgtgagcgtgcaggaatggaagttcgtgacgttcactactctcactatggccgtatgtgtccgattgaaacaccagagggtccaaacattggtttgatcaactctctatcttcatttgcaaaagtgaatcgtttcggctttattgaaacaccttaccgccgggttgatcctgaaacaggtaaagtgacaccgagaatcgattacttaactgctgatgaagaggataactacgttgtagcacaagcgaatgctatattaggtgaagatggttcgtttatcgatgataatatcattgctcgtttcagaggggaaaacaccgttgttcctcgaaaccgtgttgactacatggacgtttcgccaaagcaggttgtttctgcagcgacagcatgtatcccattcctagaaaacgatgactctaaccgtgctctaatgggagcgaacatgcaacgtcaggctgtgcctttgatgcagccggaatcaccgattgttggtacaggtatggagtatgtatcaggtaaagactctggtgctgctgtcatctgccgttacccaggtgttgtagaacgtgttgaagcaaaaaatatttgggttcgccgctatgaagatgtcgacggacaacaagtcaaaggaaacctagacaaatacagcttgctgaaatttgtccgctctaaccaagggacttgctacaaccagcgtccaatcgtaagtgttggagatgaagtcgtaaaaggagaaatccttgcagacggtccttcaatggaaaaaggtgaattggctctaggacgtaacgttatggtcggcttcatgacttgggacggttataactacgaggatgcaatcatcatgagtgagcgccttgtaaaagatgacgtctacacatctattcatattgaagaatatgaatcagaagctcgtgatacaaagcttggaccggaagaaatcactcgcgatattccaaacgttggggaagatgctttgcgcaaccttgacgagcgtggaatcatccgtattggtgcagaagtaaaagacggagaccttcttgtagggaaagtaacgcctaaaggtgtaacagaactaacagctgaagagcgtctattacatgcaatcttcggtgaaaaggctcgtgaagtacgtgatacatctctacgtgttccacacggcggcggcggaattatccacgacgtcaaagtctttaaccgtgaagatggagatgaattacctccaggtgttaaccagttagtccgcgtatacatcgttcagaagcgtaaaatttctgaaggtgacaaaatggctggacgacatggtaacaaaggggttatctctaaaatccttccagaagaagatatgccgtatcttccagatggaacaccgattgatatcatgttaaaccctctaggggtaccatctcgtatgaacatcggtcaggtacttgagcttcatatgggtatggctgcacgttaccttggcatccacattgcgtcaccagtatttgatggtgcgcgtgaggaagatgtttgggaaacgcttgaagaagcaggtatgtcccgtgatgcgaaaacagtcctttatgacggtcgaactggtgaaccattcgataaccgtgtatcagtcggaatcatgtacatgatcaaactggctcacatggttgacgacaaacttcacgctcgttcaactggaccatactcacttgttacgcagcagccacttggcggtaaagcacagtttggtggtcagcgattcggagagatggaagtatgggcacttgaagcttacggtgcagcatacacacttcaagagatcttaacagttaaatcggatgacgtggtgggtcgtgtgaaaacatacgaagccatcgtcaaaggggataacgtccctgaaccaggtgtccctgaatcattcaaagtgttaatcaaagaacttcaaagtttaggtatggatgtcaaaatcttatctggcgatgaaaaagagatagaaatgagagatttagaagacgatgaggaaacgaagaaagcagacggattagcgttatctaatgacgaagatgctgcagacctcgcacctgtcgatcttgaacgtgacgcagtcacaaaagaatag

SEQ ID NO: 22 - DNA, 1191 bp, Bacillus pumilus
  source 1..1191: mol_type = genomic DNA
gtgaagaataaatggttcgcctattttattggcagagtggaagtggaaatcaagggaaacggcattgagcggctcatcaatgagtgcacgagacaggggatcacaatgtttcaagtgagccgccgtcaagacagcgtgcgcttatttattcgcttatcagatgtacatgccttcagaaaagtacaaagacatcatgacgtaaaatgttcatttcatcaaaagaagggatttccgttccttctcctatggtcaaggaagaatattgggtttacccttgggattgtgttctttctagtgacgatattggcgctttcaaacatggtgtggaaaattgatattaaaggagccaatccagaaactgaacatcagatgagaaagcatttagacgagattggtgtgcaaaaaggccgttttcagtttctaatgggaacacctgaaaaaattcaaaaatcactgaccgccaatattcaaagcattacatgggttggcgttgaactaaacggtacaacatttcaaatgaaagttgtggaaaaaaatgagccggaaaaagagaaatatacgagtcctcagcatattgtggccaagaagaaggcggtcatcacgagaatgtatgtggaaaaaggggagccgcttgccgcagttgatgaacatgtgaagaaaggacaaatgctcgtctctggcctcatcggcagcgaagaccagcaaaaaacggttggtgctaaagcgaaaatttatggtgaaacgtggtatcgttctgaagtttctgtccctcttcgaacatcttttgatgtctttacgggtaaaatgaagacaaagcacaagctctccgcatttggaggttcaatgccattttggggcttttcctttaaaaaggatgattttaagcagccaaaaacagaaactgaagttcacccactccatttcttaaacttccagctcccattttcctatgaaaaagaaacgacacgcgaaagcgaaaaaataaaccggacatacacaaataaagaagcggttcaagcagggattaaaatgggtaaaaaagaattagaagagaagctaggtcaaacaggagaggtgaaaagtgaaaaagttttgcacgaggcaacagggaatggtaaagttaagttaatcatcctttaccaagtaatagaagatattgttcaaccaacacctattgttcagggagactag

SEQ ID NO: 23 - DNA, 1456 bp, Bacillus pumilus
  source 1..1456: mol_type = genomic DNA
gttagcggcggacgggtgagtaacacgtgggtaacctgcctgtaagactgggataactccgggaaaccggagctaataccggatagttccttgaaccgcatggttcaaggatgaaagacggtttcggctgtcacttacagatggacccgcggcgcattagctagttggtggggtaatggctcaccaaggcgacgatgcgtagccgacctgagagggtgatcggccacactgggactgagacacggcccagactcctacgggaggcagcagtagggaatcttccgcaatggacgaaagtctgacggagcaacgccgcgtgagtgatgaaggttttcggatcgtaaagctctgttgttagggaagaacaagtgcgagagtaactgctcgcaccttgacggtacctaaccagaaagccacggctaactacgtgccagcagccgcggtaatacgtaggtggcaagcgttgtccggaattattgggcgtaaagggctcgcaggcggtttcttaagtctgatgtgaaagcccccggctcaaccggggagggtcattggaaactgggaaacttgagtgcagaagaggagagtggaattccacgtgtagcggtgaaatgcgtagagatgtggaggaacaccagtggcgaaggcgactctctggtctgtaactgacgctgaggagcgaaagcgtggggagcgaacaggattagataccctggtagtccacgccgtaaacgatgagtgctaagtgttagggggtttccgccccttagtgctgcagctaacgcattaagcactccgcctggggagtacggtcgcaagactgaaactcaaaggaattgacgggggcccgcacaagcggtggagcatgtggtttaattcgaagcaacgcgaagaaccttaccaggtcttgacatcctctgacaaccctagagatagggctttcccttcggggacagagtgacaggtggtgcatggttgtcgtcagctcgtgtcgtgagatgttgggttaagtcccgcaacgagcgcaacccttgatcttagttgccagcatttagttgggcactctaaggtgactgccggtgacaaaccggaggaaggtggggatgacgtcaaatcatcatgccccttatgacctgggctacacacgtgctacaatggacagaacaaagggctgcgagaccgcaaggtttagccaatcccataaatctgttctcagttcggatcgcagtctgcaactcgactgcgtgaagctggaatcgctagtaatcgcggatcagcatgccgcggtgaatacgttcccgggccttgtacacaccgcccgtcacaccacgagagtttgcaacacccgaagtcggtgaggtaacctttatggagccagccgccgaaggtggggcagatgattggggtgaagtcgtaacaaggtagccgtatcggaaggtgcggctggatcacctccttt

SEQ ID NO: 24 - DNA, 1626 bp, Bacillus pumilus
  source 1..1626: mol_type = genomic DNA
atggcaaaagatattaagttcagtgaagaagcacgtcgcgcgatgttacgtggtgtagatgcacttgcagatgctgtaaaagtaactttaggacctaaaggacgtaacgtggttcttgagaaaaaattcggttctccacttatcacaaatgatggtgtgacgatcgcaaaagaaatcgaattagaagatgcatttgaaaacatgggtgcaaaacttgtggctgaagttgcaagcaaaacaaacgacgtagctggtgacggtacaacgactgcaacagttctagctcaagcgatgatccgtgaaggtcttaaaaacgtaacagctggtgcaaaccctgttggcgttcgtaaagggatcgaagaagcagtgaaagtagcacttgaaggcttgcacgagatttctaaaccaatcgaaggcaaagaatcaattgctcaagtagcgtctatttctgcagcagatgaagaagtgggaagcctaatcgctgaagcaatggagcgtgtaggtaacgacggcgtgatcacaatcgaagaatctaaaggattcacaactgagcttgaagtagttgaaggaatgcagtttgaccgcggatatgcttcaccatacatggtgacggattctgataagatggaagcggttcttgaaaatccttacatcttaatcactgataaaaaaatcacgaacattcaagaaatccttcctgtacttgagcaagttgtacaacaaggaaaaccattgttgatcattgctgaagatgtagaaggcgaagcacttgcaacacttgttgtaaacaaacttcgtggaacattcaacgcagtggcagtaaaagcacctggattcggtgatcgtcgtaaagcaatgcttgaagacatctctgttctaactggcggagagttaatcacagaagacctaggacttgacctgaaatcaactgaaatcggtcagcttggccgcgcgtctaaagtcgttgtgacaaaagaaaacacaacgatcgtagaaggttcaggagattctgctcaaatcgcagcacgcgtgaaccaaatccgtgcgcaagttgaagaaacaacttctgaattcgataaagaaaaattacaagaacgtcttgctaaactagctggtggcgtcgcagtcatcaaagttggtgctgcaactgaaacagaactaaaagagcgtaaactacgcatcgaggatgccttgaactcaactcgtgcagcagttgaagaaggtatcgtatccggtggtggtacagcacttgtgaatgtatacaaaaaagtcgcttcaatcgaagcagatggtgacgttcaaactggtgtgaacatcgttctacgttctcttgaagagccaatccgtcaaatcgctcacaacgcaggtcttgaaggatcagtcatcgttgagcgcttgaaaaacgaagaaattggcgtaggcttcaacgcagcaacaaacgaatgggtaaacatgattgaaaaaggaatcgttgacccaacaaaagtaactcgctctgcacttcaaaacgcagcttctgttgcagcaatgcttctaacaactgaagcagtcgttgctgacaaaccagaagaaggcggctcaggcggcggaatgccggatatgggcggcatgggtggcatgatgtaa

SEQ ID NO: 25 - DNA, 1917 bp, Bacillus pumilus
  source 1..1917: mol_type = genomic DNA
atggaacagcaacataatagttatgatgaaaatcagatacaggtgcttgaaggactagaagctgttagaaaacgtccaggaatgtacattgggtcaaccagtgcaaaaggacttcaccatcttgtatgggaaattgtcgacaacagtattgatgaggctttagctggatattgcacagatattacggtgcaaattgaaaaggataatagcattacagtgaaagataatggccgcggaattcctgttgggattcatgagaaaatgggacgtcctgctgtagaggttattatgactgttcttcacgctggcggtaaatttgacggcagcggttataaagtatctggcggtctgcatggcgtaggggcatctgttgttaatgcgttatctacgaccttagacgtgaccgtatatcgtgatgggaaaattcattatcaacaattcaaacgcggtgttccagttggagatttaaagatcattggtgaaacagatgttacagggacaaccactcattttgtgccagatacagaaatttttactgaaaccattgaatttgattacgacacacttgccaaccgtgtacgtgagttagctttcttaacaaaaggtgtcaacatcgttattgaagatttacgtgaggggaaagaacgacgaaatgaatactgctatgaaggcggtattaagagctatgtagaacatttaaatcgctcaaaagaagtcgttcatgaagaacccgtttacattgaaggtgaaaaagatggaatcacggttgaagtggcattacaatataacgattcctatacaagcaacatctattccttcgccaacaatatcaacacgtatgaaggcggaacacacgaagcaggctttaaaacagggctgacgcgtgtcatcaatgattatgctcgtaaaaatggcgtattcaaagatggagactcgaatttgagcggtgaagatgtgcgagaaggcttaacagccattatctccatcaaacatccaaatcctcaattcgaaggacaaacgaagacaaagcttgggaactcagaagcaagaaccattaccgactcccttttctctgaagcacttgagaaattcctcttagagaaccctgatgctgcaaagaaaattgtggagaaaggcgtgatggcagctcgtgcaagaatggctgccaaaaaggcacgtgagctgacaagacgtaaaagtgcactggaagtctccagcttaccagggaaactggcggactgttcatctaaagacccttccatctctgaactttatatcgtagagggagattctgcgggcggatctgctaagcaaggccgtgatcgtcacttccaagcgatcttaccgttaagagggaagatcttaaacgttgaaaaagcgcgattagataaaattctatcgaacaacgaagttcgttctatgattacagcgttaggaactggaatcggtgaagacttcactttagagaaagctcgctatcacaaagttgtgatcatgacggatgcggatgtcgatggtgcccatattcgcacgctgctcttaacgttcttctatcgctacatgcgtgaaatcattgaaaacggttatgtgtatattgcgcagccacctttatttaaagtgcagcaaggtaaacgtgttgagtatgtgtataacgataaacagctagatgagctgctaaagacattgcctcaaacaccaaaacctggacttcagcgctataaaggtcttggagaaatgaacgcaactcagctttgggaaacaacaatggaccctgatgcgagaacacttcttcaagtcacacttgaggatgcgatcgatgctgatgagacatttgaaatgctcatgggagataaagtagagccgagaagaaactttatcgaagaaaatgcgcaatacgtgaaaaacctcgatatttag

SEQ ID NO: 26 - DNA, 3582 bp, Bacillus pumilus
  source 1..3582: mol_type = genomic DNA
ttgacaggtcaactagttcagtatggacgacaccgccagcgcagaagctacgcacgcataagcgaagtgttagaattaccaaatctcattgaaattcaaacctcttcttatcagtggtttcttgatgagggtcttagagagatgtttcaagatatatccccaattgaggattttactggtaacctttctcttgaattcattgattacagcctaggggatcctaagtatcctgtagcagaatcaaaagaacgtgatgtaacttactctgctccactaagagtgaaagttcgtttaattaacaaagaaactggagaagtaaaagaccaagatgtgttcatgggtgatttcccaatcatgacagacacaggtacttttatcattaacggtgcggaacgtgtaatcgtttctcagttagtacgttctccaagtgtatatttcagtggtaaagtagacaaaaacggtaaaaaaggttttactgcgactgtcattccaaaccgtggcgcatggttagaatacgaaactgatgcgaaggatgtagtctatgtacgcatcgatcgcacacgtaagttgccggttacggttcttttgcgtgctctcggcttcagctctgatcaagagattcttgacctcattggcgagaatgaatacttacgcaacacgctggaaaaagacaatacagagaatgcggataaagcacttctcgaaatctacgagcgcctccgtcctggagagccgccaactgttgaaaatgcgaaaagcctgctagactctcgcttcttcgatccgaagagatatgacctagcaaatgttggacgctacaagattaataaaaagcttcatattaaaaatagactgttcaatcaaaaattggctgaaacgttagttgaccctgaaacaggtgaaattctagcagaaaaaggtcaaattttagacagaagagttcttgataaagttcttccatacttagaaaacggcatcggatttagaaagctttatccaaatggtggcgtagtagaagatgaagtagaacttcaatctattaagatttatgcaccgtctgatcaagaaggcgagcaagtgatcaacgtgatcgggaatgcatacgtagaggaagctgtgaaaaacatcacgccttctgacatcattgcatcgatcagttacttcttcaaccttcttcatggtgtaggtgacacagatgatatcgatcaccttggtaaccgtcgcctgcgttctgtaggtgagcttctgcaaaaccaattccgtattggtttaagcagaatggagcgtgttgttcgtgaaagaatgtcgatccaagacacaaacacgatcacacctcagcaactgatcaacatccgtcctgtgatcgcttctatcaaagagttctttggtagctctcagctttctcagttcatggatcaaacaaacccgcttgctgaattgacgcacaaacgtcgtctgtcagcgcttgggcctggtggtttgacacgtgagcgtgcaggaatggaagttcgtgacgttcactactctcactatggccgtatgtgtccgattgaaacaccagagggtccaaacattggtttgatcaactctctatcttcatttgcaaaagtgaatcgtttcggctttattgaaacaccttaccgccgggttgatcctgaaacaggtaaagtgacaccgagaatcgattacttaactgctgatgaagaggataactacgttgtagcacaagcgaatgctatattaggtgaagatggttcgtttatcgatgataatatcattgctcgtttcagaggggaaaacaccgttgttcctcgaaaccgtgttgactacatggacgtttcgccaaagcaggttgtttctgcagcgacagcatgtatcccattcttagaaaacgatgactctaaccgtgctctaatgggagcgaacatgcaacgtcaggctgtgcctttgatgcagccagaatcaccgattgttggtacaggtatggagtatgtatcaggtaaagactctggtgctgctgtcatctgccgttacccaggtgttgtagaacgtgttgaagcaaaaaatatttgggttcgccgctatgaagatgtcgacggacaacaagtcaaaggaaacctagacaaatacagcttgctgaaatttgtccgctctaaccaagggacttgctacaaccagcgtccaatcgtaagtgttggagatgaagtcgtaaaaggagaaatccttgcagacggtccttcaatggaaaaaggtgaattggctctaggacgtaacgttatggtcggcttcatgacttgggacggttataactacgaggatgcgatcatcatgagtgagcgccttgtaaaagatgacgtctacacatctattcatattgaagaatatgaatcagaagctcgtgatacaaagcttggaccggaagaaatcactcgtgatattccaaacgttggggaagatgctttgcgcaaccttgacgagcgtggaatcatccgtattggtgcagaagtaaaagacggagaccttcttgtagggaaagtaacgcctaaaggtgtaacagaactaacagctgaagaacgtctattacatgcaatcttcggtgaaaaggctcgtgaagtacgtgatacatctctacgtgttccacacggcggcggcggaattatccacgacgtcaaagtctttaaccgtgaagatggagatgaattacctccaggtgttaaccagttagtccgcgtatacatcgttcagaagcgtaaaatttctgaaggtgacaaaatggctggacgacatggtaacaaaggggttatctctaaaatccttccagaagaagatatgccgtatcttccagatggaacaccgattgatatcatgttaaaccctctaggggtaccatctcgtatgaacatcggtcaggtacttgagcttcatatgggtatggctgcacgttaccttggcatccacattgcgtcaccagtatttgatggtgcgcgtgaggaagatgtttgggaaacgcttgaagaagcaggtatgtcccgtgatgcgaaaacagtcctttatgacggtcgaactggtgaaccattcgataaccgtgtatcagtcggaatcatgtacatgatcaaactggctcacatggttgacgacaaacttcacgctcgttcaactggaccatactcacttgttacgcagcagccacttggcggtaaagcacagtttggtggtcagcgtttcggagagatggaagtatgggcacttgaagcttacggtgcagcatacacacttcaagagatcttaacagttaaatcggatgacgtggtgggtcgtgtgaaaacatacgaagccatcgtcaaaggggataacgtccctgaaccaggtgtccctgaatcattcaaagtgttaatcaaagaacttcaaagtttaggtatggatgtcaaaatcctatctggcgatgaagaagagatagaaatgagagatttagaagacgatgaggaaacgaagaaagcagacggattagcgttatctaatgacgaagatgctgcagacctcgcacctgtcgatcttgaacgtgacgcagtcacaaaagaatag

SEQ ID NO: 27 - DNA, 1191 bp, Bacillus pumilus
  source 1..1191: mol_type = genomic DNA
gtgaagaataaatggttcgcctattttattggcagagtggaagtggaaatcaagggaaacggcattgagcggctcatcaatgagtgcacgagacaggggatcacaatgtttcaagtgagccgccgtcaagacagcgtgcgcttatttattcgcttatcagatgtacatgccttcagaaaagtacaaagacatcatgaggtaacatgttcatttcatcaaaagaagggatttccgttccttctcctatggtcaaggaagaatattgggtttacccttgggattgtgttctttctagtgacgatattggcactttcaaacatggtgtggaaaattgatattaaaggagccaatccagaaactgaacatcagatgagaaagcatttagacgagattggtgtgcaaaaaggccgttttcagtttctaatgggaacacctgaaaaaattcaaaaatcactgaccgccaatattcaaagcataacatgggttggcgttgaactaaacggtacaacatttcaaatgaaagttgtggaaaaaaatgagccggaaaaagagaaatatacgagtcctcagcatattgtggccaagaagaaggcggtcatcacgagaatgtatgtggaaaaaggggagccgcttgccgcagttgatgaacatgtgaagaaaggacaaatgctcgtctctggcctcattggcagcgaagaccagcaaaaaacggttggtgctaaagcgaaaatttatggtgaaacgtggtatcgttctgaagtttctgtccctcttcgaacatcttttgatgtctttacgggtaaaatgaagacaaagcacaagctctccgcatttggaggttcaatgccattttggggcttttcctttaaaaaagatgattttaagcagccaaaaacagaaactgaagttcacccactccatttcttaaacttccagctcccattttcctatgaaaaagaaacgacacgcgaaagcgaaaaaataaaccggacatacacaaataaagaagcggttcaagcagggattaaaatgggtaaaaaagaattagaagagaagctaggtcaaacaggagaggtgaaaagtgaaaaagttttgcacgaggcaacagggaatggtaaagttaagttaatcatcctttaccaagtaatagaagatattgttcaaccaacacctattgttcagggagactag

SEQ ID NO: 28 - DNA, 1456 bp, Bacillus pumilus; identical to SEQ ID NO: 18
  source 1..1456: mol_type = genomic DNA

SEQ ID NO: 29 - DNA, 1635 bp, Bacillus pumilus
  source 1..1635: mol_type = genomic DNA
atggcaaaagatattaagttcagtgaagaagcacgtcgcgcgatgttacgtggtgtagatgcacttgcagatgctgtaaaagtaactttaggacctaaaggacgtaacgtggttcttgagaaaaaattcggttctccacttatcacaaatgatggtgtgacgatcgcaaaagaaatcgaattagaagatgcatttgaaaacatgggtgcaaaacttgtggctgaagttgcaagcaaaacaaacgacgtagctggtgacggtacaacgactgcaacagttctagctcaagcgatgatccgtgaaggtcttaaaaacgtaacagctggtgcaaaccctgttggtgtacgtaaagggatcgaagaagcagtgaaagtagctcttgaaggcttgcacgagatttctaaaccaatcgaaggcaaagaatcaattgctcaagttgcgtctatttctgcagcagatgaagaagtgggaagccttatcgctgaagcaatggagcgtgtaggtaacgacggcgtcatcactatcgaagaatctaaaggtttcacaactgagctagaagtggttgaaggaatgcagtttgaccgcggatatgcttcaccatacatggtgacggattctgataagatggaagcggttcttgaaaatccttacatcttaatcactgataaaaaaattacaaacattcaagaaatccttcctgtactcgagcaagttgtacaacaaggaaaaccattgttgatcattgcagaagatgtagaaggcgaagcacttgcaacacttgttgtaaacaaacttcgtggaacattcaacgcagtggcagtaaaagcacctggattcggtgatcgtcgtaaagcaatgcttgaagacatctctgttctaactggcggagagttaatcacagaagacctaggacttgacctgaaatcaactgaaatcggtcagcttggccgcgcgtctaaagtcgttgtgacaaaagaaaacacaacgatcgtagaaggctcaggagattctgctcaaatcgcagcacgcgtgaaccaaatccgtgcgcaagttgaagaaacaacttctgaattcgataaagaaaaattacaagaacgtcttgctaaactagctggtggcgtcgctgtcatcaaagttggtgctgcaactgaaacagaactaaaagagcgtaaactacgcatcgaggatgccttgaactcaactcgtgcagcagttgaagaaggtatcgtatccggtggtggtacagcacttgtgaatgtatacaaaaaagtcgcttcaatcgaagcagatggtgacgttcaaactggtgtgaacatcgttctacgttctcttgaagagccaatccgtcaaatcgctcacaacgcaggtcttgaaggatcagtcatcgttgagcgcttgaaaaacgaagaaattggagtaggcttcaacgcagcaacaaacgaatgggtaaacatgattgaaaaaggaatcgttgacccaacaaaagtaactcgctctgcacttcaaaacgcagcttctgttgcagcaatgcttctaacaactgaagcagtcgttgctgacaaaccagaagaaggcggctcaggcggcggaatgccggatatgggcggcatgggcggaatgggtggcatgatgtaa

SEQ ID NO: 30 - DNA, 1917 bp, Bacillus pumilus
  source 1..1917: mol_type = genomic DNA
atggaacagcaacataatagttatgatgaaaatcagatacaggtgcttgaaggactagaagctgttagaaaacgtccaggaatgtacattgggtcaaccagtgcaaaaggacttcaccatcttgtatgggaaattgtcgacaacagtattgatgaggctttagctggatattgcacagatattacggtgcaaattgaaaaggataatagcattacagtgaaagataatggccgcggaattcctgttgggattcatgagaaaatgggacgtcctgctgtagaggttattatgactgttcttcacgctggcggtaaatttgacggcagcggttataaagtatctggcggtctgcatggcgtaggggcatctgttgttaatgcgttatctacgaccttagacgtgaccgtatatcgtgatgggaaaattcattatcaacaattcaaacgcggtgttccagttggagatttaaagatcattggtgaaacagatgttacagggacaaccactcattttgtgccagatacagaaatttttactgaaaccattgaatttgattacgacacacttgccaaccgtgtacgtgagttagctttcttaacaaaaggtgttaacatcgttattgaagatttacgtgaggggaaagaacgacgaaatgaatactgctatgaaggcggtattaagagctatgtagaacatttaaatcgctcaaaagaagtcgttcatgaagaacccgtttacattgaaggtgaaaaagatggaatcacggttgaagtggcattacaatataacgattcctatacaagcaacatctattccttcgccaacaatatcaacacgtatgaaggcggaacacacgaagcaggctttaaaacagggctgacgcgtgtcatcaatgattatgctcgtaaaaatggcgtattcaaagatggagactcgaatttaagcggtgaagatgtgcgagaaggcttaacagccattatctccatcaaacatccaaatcctcaattcgaaggacaaacgaagacaaagcttgggaactcagaagcaagaaccattaccgactcccttttctctgaagcacttgagaaattcctcttagagaaccctgatgctgcaaagaaaattgtggagaaaggcgtgatggcagctcgtgcaagaatggctgccaaaaaggcacgtgagctgacaagacgtaaaagtgcactggaagtctccagcttaccggggaaactggcggactgttcttctaaagacccttccatctctgaactttatatcgtagagggagattctgcgggcggatctgctaagcaaggccgtgatcgtcacttccaagcgatcttaccgttaagagggaagatcttaaacgttgaaaaagcgcgattagataaaattctatcgaacaacgaagttcgttctatgattacagcgttaggaactggaatcggtgaagacttcactttagagaaagctcgctatcacaaagttgtgatcatgacggatgcggatgtcgatggtgcccatattcgcacgctgctcttaacgttcttctatcgctacatgcgtgaaatcattgaaaacggttatgtgtatattgcgcagccacctttatttaaagtgcagcaaggtaaacgtgttgagtatgtgtataacgataaacagctagatgagctgctaaagacattgcctcaaacaccaaaacctggacttcagcgctataaaggtcttggagaaatgaacgcaactcagctttgggaaacaacaatggatcctgatgcgagaacacttcttcaagtgacgcttgaggatgcgattgatgctgatgagacatttgaaatgttgatgggagataaagtagaaccgagacgaaactttatcgaagaaaatgcacaatacgtgaaaaatcttgatatttag

SEQ ID NO: 31 - DNA, 3582 bp, Bacillus pumilus; identical to SEQ ID NO: 26
  source 1..3582: mol_type = genomic DNA

SEQ ID NO: 32 - DNA, 1191 bp, Bacillus pumilus
  source 1..1191: mol_type = genomic DNA
gtgaagaataaatggttcgcctattttattggcagagtggaagtggaaatcaagggaaacggcattgagcggctcatcaatgagtgcacgagacaggggatcacaatgtttcaagtgagccgccgtcaagacagcgtgcgcttatttattcgcttatcagatgtacatgccttcagaaaagtacaaagacatcatgaggtaacatgttcatttcatcaaaagaagggatttccgttccttctcctatggtcaaggaagaatattgggtttacccttgggattgtgttctttctagtgacgatattggcactttcaaacatggtgtggaaaattgatattaaaggagccaatccagaaactgaacatcagatgagaaagcatttagacgagattggtgtgcaaaaaggccgtttccagtttctaatgggaacacctgaaaaaattcaaaaatcactgaccgccaatattcaaagcataacatgggttggcgttgaactaaacggtacaacatttcaaatgaaagttgtggaaaaaaatgagccggaaaaagagaaatatacgagtcctcagcatattgtggccaagaagaaggcggtcatcacgagaatgtatgtggaaaaaggggagccgcttgccgcagttgatgaacatgtgaagaaaggacaaatgctcgtctctggcctcatcggcagcgaagaccagcaaaaaacggttggtgctaaagcgaaaatttatggtgaaacgtggtatcgttctgaagtttctgtccctcttcgaacatcttttgatgtctttacgggtaaaatgaagacaaagcacaagctctccgcatttggaggttcaatgccattttggggcttttcctttaaaaaggatgattttaagcagccaaaaacagaaactgaagttcacccactccatttcttaaacttccagctcccattttcctatgaaaaagaaacgacacgcgaaagcgaaaaaataaaccggacatacacaaataaagaagcggttcaagcagggattaaaatgggtaaaaaagaattagaagagaagctaggtcaaacaggagaggtgaaaagtgaaaaagttttgcacgaggcaacagggaatggtaaagttaagttaatcatcctttaccaagtaatagaagatattgttcaaccaacacctattgttcagggagactag

SEQ ID NO: 33 - DNA, 1456 bp, Bacillus pumilus; identical to SEQ ID NO: 18
  source 1..1456: mol_type = genomic DNA

SEQ ID NO: 34 - DNA, 1635 bp, Bacillus pumilus
  source 1..1635: mol_type = genomic DNA
atggcaaaagatattaagttcagtgaagaagcacgtcgcgcgatgttacgtggtgtagatgcacttgcagatgctgtaaaagtaactttaggacctaaaggacgtaacgtggttcttgagaaaaaattcggttctccacttatcacaaatgatggtgtgacgatcgcaaaagaaatcgaattagaagatgcatttgaaaacatgggtgcaaaacttgtggctgaagttgcaagcaaaacaaacgacgtagctggtgacggtacaacgactgcaacagttctagctcaagcgatgatccgtgaaggtcttaaaaacgtaacagctggtgcaaaccctgttggcgttcgtaaagggatcgaagaagcagtgaaagtagcacttgaaggcttgcacgagatttctaaaccaatcgaaggcaaagaatcaattgctcaagtagcgtctatttctgcagcagatgaagaagtgggaagcctaatcgctgaagcaatggagcgtgtaggtaacgacggcgtgatcacaatcgaagaatctaaaggattcacaactgagcttgaagtagttgaaggaatgcagtttgaccgcggatatgcttcaccatacatggtgacggattctgataagatggaagcggttcttgaaaatccttacatcttaatcactgataaaaaaatcacgaacattcaagaaatccttcctgtacttgagcaagttgtacaacaaggaaaaccattgttgatcattgctgaagatgtagaaggcgaagcacttgcaacacttgttgtgaacaaacttcgtggaacattcaacgcagtggcagtaaaagcacctggattcggtgatcgtcgtaaagcaatgcttgaagacatctctgttctaactggcggagagttaatcacagaagacctaggacttgacctaaaatcaactgaaatcggtcagcttggccgcgcgtctaaagtcgttgtgacaaaagaaaacacaacgatcgtagaaggctcaggagattctgctcaaatcgcagcacgcgtgaaccaaatccgtgcgcaagttgaagaaacaacttctgaattcgataaagaaaaattacaagaacgtcttgctaaactagctggtggcgtcgctgtcatcaaagttggtgctgcaactgaaacagaactaaaagagcgtaaactacgcatcgaggatgccttgaactcaactcgtgcagcagttgaagaaggtatcgtatccggtggtggtacagcacttgtgaatgtatacaaaaaagtcgcttcaatcgaagcagatggtgacgttcaaactggtgtgaacatcgttctacgttctcttgaagagccaatccgtcaaatcgctcacaacgcaggtcttgaaggatcagtcatcgttgagcgcttgaaaaacgaagaaattggcgtaggcttcaacgcagcaacaaacgaatgggtaaacatgatcgaaaaaggaatcgttgacccaacaaaagtaactcgctctgcacttcaaaacgcagcttctgttgcagcaatgcttctaacaactgaagcagtcgttgctgacaaaccagaagaaggcggctcaggcggcggaatgccggatatgggcggcatgggcggaatgggtggcatgatgtaa

SEQ ID NO: 35 - DNA, 1917 bp, Bacillus pumilus
  source 1..1917: mol_type = genomic DNA
atggaacagcaacataatagttatgatgaaaatcagatacaggtgcttgaaggactagaagctgttagaaaacgtccaggaatgtacattgggtcaaccagtgcaaaaggacttcaccatcttgtatgggaaattgtcgacaacagtattgatgaggctttagctggatattgcacagatattacggtgcaaattgaaaaggataatagcattacagtgaaagataatggccgcggaattcctgttgggattcatgagaaaatgggacgtcctgctgtagaggttattatgactgttcttcacgctggcggtaaatttgacggcagcggttataaagtatctggcggtctgcatggcgtaggggcatctgttgttaatgcgttatctacgaccttagacgtgaccgtatatcgtgatgggaaaattcattatcaacaattcaaacgcggtgttccagttggagatttagagatcattggtgaaacagatgttacagggacaaccactcattttgtgccagatacagaaatttttactgaaaccattgaatttgattacgacacacttgccaaccgtgtacgtgagttagctttcttaacaaaaggtgtcaacatcgttattgaagatttacgtgaggggaaagaacgacgaaatgaatactgctatgaaggcggtattaagagctatgtagaacatttaaatcgctcaaaagaagtcgttcatgaagaacccgtttacattgaaggtgaaaaagatggaatcacggttgaagtggcattacaatataacgattcctatacaagcaacatctattccttcgccaacaatatcaacacgtatgaaggcggaacacacgaagcaggctttaaaacagggctgacgcgtgtcatcaatgattatgctcgtaaaaatggcgtattcaaagatggagactcgaatttgagcggtgaagatgtgcgagaaggcttaacagccattatctccatcaaacatccaaatcctcaattcgaaggacaaacgaagacaaagcttgggaactcagaagcaagaaccattaccgactcccttttctctgaagcacttgagaaattcctcttagagaaccctgatgctgcaaagaaaattgtggagaaaggcgtgatggcagctcgtgcaagaatggctgccaaaaaggcacgtgagctgacaagacgtaaaagtgcactggaagtctccagcttaccagggaaactggcggactgttcttctaaagacccttccatctctgaactttatatcgtagagggagattctgcgggcggatctgctaagcaaggccgtgatcgtcacttccaagcgatcttaccgttaagagggaagatcttaaacgttgaaaaagcgcgactagataaaattctatcgaacaacgaagttcgttctatgattacagcgttaggaactggaatcggtgaagacttcactttagagaaagctcgctatcacaaagttgtgatcatgacggatgcggatgtcgatggtgcccatattcgcacgctgctcttaacgttcttctatcgctacatgcgtgaaatcattgaaaacggttatgtgtatattgcgcagccacctttatttaaagtgcagcaaggtaaacgtgttgagtatgtgtataacgataaacagctagatgagctgctaaagacattgcctcaaacaccaaaacctggacttcagcgctataaaggtcttggagaaatgaacgcaactcagctttgggaaacaacaatggatcctgatgcgagaacacttcttcaagtgacgcttgaggatgcgattgatgctgatgagacatttgaaatgttgatgggagataaagtagaaccgagacgaaactttatcgaagaaaatgcacaatacgtgaaaaatcttgatatttag

SEQ ID NO: 36 - DNA, 3582 bp, Bacillus pumilus
  source 1..3582: mol_type = genomic DNA
ttgacaggtcaactagttcagtatggacgacaccgccagcgcagaagctacgcacgcataagcgaagtgttagaattaccaaatctcattgaaattcaaacctcttcttatcagtggtttcttgatgagggtcttagagagatgtttcaagatatatccccaattgaggattttactggtaacctttctcttgaattcattgattacagcctaggggatcctaagtatcctgtagcagaatcaaaagaacgtgatgtaacttactctgctccactaagagtgaaagttcgtttaattaacaaagaaactggagaagtaaaagaccaagatgtgttcatgggtgatttcccaatcatgacagacacaggtacttttatcattaacggtgcggaacgtgtaatcgtttctcagttagtacgttctccaagtgtatatttcagtggtaaagtagacaaaaacggtaaaaaaggttttactgcgactgtcattccaaaccgtggcgcatggttagaatacgaaactgatgcgaaggatgtagtctatgtacgcatcgatcgcacacgtaagttgccggttacggttcttttgcgtgctctcggcttcagctctgatcaagagattcttgacctcattggcgagaatgaatacttacgcaacacgctggaaaaagacaatacagagaatgcggataaagcacttctcgaaatctacgagcgcctccgtcctggagagccgccaactgttgaaaatgcgaaaagcctgctagactctcgcttcttcgatccgaagagatatgacctagcaaatgttggacgctacaagattaataaaaagcttcatattaaaaatagactgttcaatcaaaaattggctgaaacgttagttgaccctgaaacaggtgaaattctagcagaaaaaggtcaaattttagacagaagagttcttgataaagttcttccatacttagaaaacggcatcggatttagaaagctttatccaaatggtggcgtagtagaagatgaagtagaacttcaatctattaagatttatgcaccgtccgatcaagaaggcgagcaagtgatcaacgtgatcgggaatgcatacgtagaggaagctgtgaaaaacatcacgccttctgacatcattgcatcgattagttacttcttcaaccttcttcatggtgtaggtgacacagatgatatcgatcaccttggtaaccgtcgcctgcgttctgtaggtgagcttctgcaaaaccaattccgtattggtttaagcagaatggagcgtgttgttcgtgaaagaatgtcgatccaagacacaaacacgatcacacctcagcaactgatcaacatccgtcctgtgatcgcttctatcaaagagttctttggtagctctcagctttctcagttcatggatcaaacaaacccgcttgctgaattgacgcacaaacgtcgtctgtcagcgcttgggcctggtggtttgacacgtgagcgtgcaggaatggaagttcgtgacgttcactactctcactatggccgtatgtgtccgattgaaacaccagagggtccaaacattggtttgatcaactctctatcttcatttgcaaaagtgaatcgtttcggctttattgaaacaccttaccgccgggttgatcctgaaacaggtaaagtgacaccgagaatcgattacttaactgctgatgaagaggataactacgttgtagcacaagcgaatgctatattaggtgaagatggttcgtttatcgatgataatatcattgctcgtttcagaggggaaaacaccgttgttcctcgaaaccgtgttgactacatggacgtttcgccaaagcaggttgtttctgcagcgacagcatgtatcccattcctagaaaacgatgactctaaccgtgctctaatgggagcgaacatgcaacgtcaggctgtgcctttgatgcagccagaatcaccgattgttggtacaggtatggagtatgtatcaggtaaagactctggtgctgctgtcatctgccgttacccaggtgttgtagaacgtgttgaagcaaaaaatatttgggttcgccgctatgaagatgtcgacggacaacaagtcaaaggaaacctagacaaatacagcttgctgaaatttgtccgctctaaccaagggacttgctacaaccagcgtccaatcgtaagtgttggagatgaagtcgtaaaaggagaaatccttgcagacggtccttcaatggaaaaaggtgaattggctctaggacgtaacgtcatggtcggcttcatgacttgggacggttataactacgaggatgcgatcatcatgagtgagcgccttgtaaaagatgacgtctacacatctattcatattgaagaatatgaatcagaagctcgtgatacaaagcttggaccggaagaaatcactcgtgatattccaaacgttggggaagatgctttgcgcaaccttgacgagcgtggaatcatccgtattggtgcagaagtaaaagacggagaccttcttgtagggaaagtaacgcctaaaggtgtaacagaactaacagctgaagaacgtctattacatgcaatcttcggtgaaaaggctcgtgaagtacgtgatacatctctacgtgttccacacggcggcggcggaattatccacgacgtcaaagtctttaaccgtgaagacggagatgaattacctccaggtgttaaccagttagtccgcgtatacatcgttcagaagcgtaaaatttctgaaggtgacaaaatggctggacgacatggtaacaaaggggttatctctaaaatccttccagaagaagatatgccgtatcttccagatggaacaccgattgatatcatgttaaaccctctaggggtaccatctcgtatgaacatcggtcaggtacttgagcttcatatgggtatggctgcacgttaccttggcatccacattgcgtcaccagtatttgatggtgcgcgtgaggaagatgtttgggaaacgcttgaagaagcaggtatgtcccgtgatgcgaaaacagtcctttatgacggtcgaactggtgaaccattcgataaccgtgtatcagtcggaatcatgtacatgatcaaactggctcacatggttgacgacaaacttcacgctcgttcaactggaccatactcacttgttacgcagcagccacttggcggtaaagcacagtttggtggtcagcgtttcggagagatggaagtatgggcacttgaagcttacggtgcagcatacacacttcaagagatcttaacagttaaatcggatgacgtggtgggtcgtgtgaaaacatacgaagccatcgtcaaaggggataacgtccctgaaccaggtgtccctgaatcattcaaagtgttaatcaaagaacttcaaagtttaggtatggatgtcaaaatcctatctggcgatgaagaagagatagaaatgagagatttagaagacgatgaggaaacgaagaaagcagacggattagcgttatctaatgacgaagatgctgcagacctcgcacctgtcgatcttgaacgtgacgcagtcacaaaagaatag

SEQ ID NO: 37 - DNA, 1191 bp, Bacillus pumilus
  source 1..1191: mol_type = genomic DNA
gtgaagaataaatggttcgcctattttattggcagagtggaagtggaaatcaagggaaacggcattgagcggctcatcaatgagtgcacgagacaggggatcacaatgtttcaagtgagccgccgtcaagacagcgtgcgcttatttattcgcttatcagatgtacatgccttcagaaaagtacaaagacatcatgacgtaaaatgttcatttcatcaaaagaagggatttccgttccttctcctatggtcaaggaagaatattgggtttacccttgggattgtgttctttctagtgacgatattgtcgctttcaaacatggtgtggaaaattgatattaaaggagccaatccagaaactgaacatcagatgagaaagcatttagacgagattggtgtgcaaaaaggccgttttcagtttctaatgggaacacctgaaaaaattcaaaaatcactgaccgccaatattcaaagcataacatgggttggcgttgaactaaacggtacaacatttcaaatgaaagttgtggaaaaaaatgagccggaaaaagagaaatatacgagtcctcagcatattgtggccaagaagaaggcggtcatcacgagaatgtatgtggaaaaaggggagccgcttgccgcagttgatgaacatgtgaagaaaggacaaatgctcgtctctggcctcatcggcagcgaagaccagcaaaaaacggttggtgctaaagcgaaaatttatggtgaaacgtggtatcgttctgaagtttctgtccctcttcgaacatcttttgatgtctttacgggtaaaatgaagacaaagcacaagctctccgcatttggaggttcaatgccattttggggcttttcctttaaaaaggatgattttaagcagccaaaaacagaaactgaagttcacccactccatttcttaaacttccagctcccattttcctatgaaaaagaaacgacacgcgaaagcgaaaaaataaaccggacatacacaaataaagaagcggttcaagcagggattaaaatgggtaaaaaagaattagaagagaagctaggtcaaacaggagaggtgaaaagtgaaaaagttttgcacgaggcaacagggaatggtaaagttaagttaatcatcctttaccaagtaatagaagatattgttcaaccaacacctattgttcagggagactag

SEQ ID NO: 38 - DNA, 1456 bp, Bacillus pumilus; identical to SEQ ID NO: 18
  source 1..1456: mol_type = genomic DNA

SEQ ID NO: 39 - DNA, 1635 bp, Bacillus pumilus; identical to SEQ ID NO: 19
  source 1..1635: mol_type = genomic DNA

SEQ ID NO: 40 - DNA, 1917 bp, Bacillus pumilus; identical to SEQ ID NO: 20
  source 1..1917: mol_type = genomic DNA

SEQ ID NO: 41 - DNA, 3582 bp, Bacillus pumilus; identical to SEQ ID NO: 21
  source 1..3582: mol_type = genomic DNA

SEQ ID NO: 42 - DNA, 1191 bp, Bacillus pumilus; identical to SEQ ID NO: 22
  source 1..1191: mol_type = genomic DNA

SEQ ID NO: 43 - DNA, 1456 bp, Bacillus altitudinis
  source 1..1456: mol_type = genomic DNA
gttagcggcggacgggtgagtaacacgtgggtaacctgcctgtaagactgggataactccgggaaaccggagctaataccggatagttccttgaaccgcatggttcaaggatgaaagacggtttcggctgtcacttacagatggacccgcggcgcattagctagttggtgaggtaacggctcaccaaggcgacgatgcgtagccgacctgagagggtgatcggccacactgggactgagacacggcccagactcctacgggaggcagcagtagggaatcttccgcaatggacgaaagtctgacggagcaacgccgcgtgagtgatgaaggttttcggatcgtaaagctctgttgttagggaagaacaagtgcaagagtaactgcttgcaccttgacggtacctaaccagaaagccacggctaactacgtgccagcagccgcggtaatacgtaggtggcaagcgttgtccggaattattgggcgtaaagggctcgcaggcggtttcttaagtctgatgtgaaagcccccggctcaaccggggagggtcattggaaactgggaaacttgagtgcagaagaggagagtggaattccacgtgtagcggtgaaatgcgtagagatgtggaggaacaccagtggcgaaggcgactctctggtctgtaactgacgctgaggagcgaaagcgtggggagcgaacaggattagataccctggtagtccacgccgtaaacgatgagtgctaagtgttagggggtttccgccccttagtgctgcagctaacgcattaagcactccgcctggggagtacggtcgcaagactgaaactcaaaggaattgacgggggcccgcacaagcggtggagcatgtggtttaattcgaagcaacgcgaagaaccttaccaggtcttgacatcctctgacaaccctagagatagggctttcccttcggggacagagtgacaggtggtgcatggttgtcgtcagctcgtgtcgtgagatgttgggttaagtcccgcaacgagcgcaacccttgatcttagttgccagcattcagttgggcactctaaggtgactgccggtgacaaaccggaggaaggtggggatgacgtcaaatcatcatgccccttatgacctgggctacacacgtgctacaatggacagaacaaagggctgcgagaccgcaaggtttagccaatcccacaaatctgttctcagttcggatcgcagtctgcaactcgactgcgtgaagctggaatcgctagtaatcgcggatcagcatgccgcggtgaatacgttcccgggccttgtacacaccgcccgtcacaccacgagagtttgcaacacccgaagtcggtgaggtaacctttatggagccagccgccgaaggtggggcagatgattggggtgaagtcgtaacaaggtagccgtatcggaaggtgcggctggatcacctccttt

SEQ ID NO: 44 - DNA, 1635 bp, Bacillus altitudinis
  source 1..1635: mol_type = genomic DNA
atggcaaaagatattaagttcagtgaagaagcacgtcgtgcgatgttacgtggtgtagatgcacttgcagatgctgtaaaagtaactttaggacctaaaggacgtaacgtggttcttgagaaaaaattcggttctccacttatcacaaatgatggtgtaacgattgcaaaagaaatcgaattagaagatgcatttgaaaacatgggtgcaaaacttgtggctgaagttgcaagcaaaacaaacgatgtagctggtgacggtactactactgcaacggttctagctcaagcgatgatccgtgaaggtcttaaaaacgtaacagctggtgcaaaccctgttggcgttcgtaaaggaatcgaagaagcagtgaaagtagcacttgaaggcttgcatgagatttctaaaccaatcgaaggtaaagaatcaattgctcaagttgcgtctatttctgcagcagatgaagaagtcggcagcctaattgctgaagcgatggagcgtgtaggaaacgacggcgtcatcacaattgaagaatctaaaggtttcacaactgagcttgaagtggttgaaggaatgcagtttgaccgtggatacgcttcaccatacatggtcactgattctgataagatggaagcggttcttgaaaatccttacatcttaatcactgataaaaagatcacaaacattcaagaaatccttcctgtacttgagcaagtcgtacaacaaggaaaaccattattgatcattgctgaagatgtagaaggcgaagcacttgcaacacttgttgtgaacaaacttcgtggaacattcaacgcagtggcagtaaaagcacctggattcggtgaccgtcgtaaagcaatgcttgaagacatctctgttctaactggcggagaactcatcactgaagacctaggacttgacctgaaatcaactgaaattggtcagcttggccgtgcgtctaaagtggttgtgacaaaagaaaacacaacgatcgtagaaggctcaggagattctgctcaaatcgcagcacgtgtgaaccaaatccgtgcgcaagtagaagaaaccacttctgaattcgataaagaaaaattacaagaacgtcttgcaaaactagctggcggcgttgctgtcatcaaagttggtgctgcaactgaaacagaactaaaagaacgtaaactacgcatcgaggatgcactgaactcaactcgtgcagcagttgaagaaggtatcgtatccggtggtggtacagcacttgtgaatgtatacaacaaagtcgcttccatcgaagctgatggtgacgttcaaacaggtgtcaacatcgttctacgttctcttgaagagccaattcgtcaaatcgctcacaacgcaggtcttgaaggatcagtcatcgttgagcgcttgaaaaacgaagaaattggcgtaggcttcaacgcagcaacaaacgaatgggtaaacatgatcgaaaaaggaatcgttgacccaacaaaagtcactcgctctgcacttcaaaacgcagcttctgtagcagctatgcttcttacaactgaagcagtcgtagctgacaaaccagaagaaggcggctcaggcggcggaatgccggatatgggcggtatgggcggaatgggtggaatgatgtaa

SEQ ID NO: 45 - DNA, 1917 bp, Bacillus altitudinis
  source 1..1917: mol_type = genomic DNA
atggaacagcaacataatagttatgatgaaaatcagatacaggtgctcgaaggactagaagcggttagaaaacgtccaggaatgtacattgggtcaaccagtgcaaaaggacttcaccatcttgtatgggaaattgtcgacaacagtattgatgaggctttagctggttattgtacagacattacagtgcaaattgaaaaagataatagcatcacagtgaaagataacggccgcggaattcctgttgggattcacgaaaaaatgggacgtcctgctgtagaagtcattatgacggttcttcacgctggtggtaaatttgacggcagcggttataaagtatctggcggtctgcacggtgtaggggcatctgttgttaatgcgttatctacgaccttagacgtgaccgtataccgtgatggaaaaattcattatcaacaattcaaacgcggtgttccagttggagatttagagatcattggtgaaacagatgtaacagggacaaccactcattttgtgccagatccagaaattttcactgaaaccattgaatttgattacgacacacttgctaaccgtgtacgtgagttagctttcttaacaaaaggcgtcaacatcatcattgaagacttacgtgaaggcaaagagcgaagaaacgaatactgctatgaaggcggtattaagagctatgtagaacatttgaatcgctcgaaggaagtcgttcatgaagaaccagtttacatcgagggtgaaaaagacggaatcaccgttgaagttgcactgcaatacaacgattcctatacaagcaatatttattctttcgccaacaacatcaacacatatgaaggcggatcacacgaagctggctttaaaaccggtctgacgcgtgtcatcaatgattatgctcgtaaaaatggcgtattcaaagatggagactcgaatttgagcggagaagatgtacgagaaggcttgacagccattatctctatcaaacatccagaccctcaattcgaaggacaaacgaagacaaagctcggtaactcagaagcaagaaccattaccgactccctcttctccgaagcacttgagaaattcctcttagagaaccctgatgctgcaaagaaaattgtggagaaaggtgtgatggcagctcgtgcaagaatggctgccaaaaaggcacgtgagttgacaagacgtaaaagtgcactggaagtctctagcttgcctgggaaactggcagactgttcttctaaagatccatccatctctgagctttatatcgtagagggagactctgcgggcggatctgctaagcaaggtcgtgatcgacatttccaagcgatcttaccgttaagagggaagatcctaaacgttgaaaaagcacgactagataaaattttatctaacaacgaggttcgttcaatgattacagcgctagggactggaatcggagaagacttcactttagagaaagcacgttatcacaaaattgtgatcatgactgatgctgatgttgatggagcgcatatacggacgctactcctaacattcttctatcgctacatgcgtgaaatcattgaaaacggttatgtgtatattgcacagccgcctttatataaagtacagcaaggaaaacgtgttgaatacgtgtataacgataaacagctagatgaactgttaaaaacgctgcctcaaacaccgaaacctggacttcagcgttataaaggtcttggagagatgaatgctactcagctttgggaaacaacaatggatcctgatgcgagaacacttcttcaagttacacttgaggatgcaatcgatgctgatgagacttttgaaatgctaatgggagataaagtagagccgagacgtaactttatcgaagaaaatgcacaatacgtaaaaaatcttgatatttag

SEQ ID NO: 46 - DNA, 3582 bp, Bacillus altitudinis
  source 1..3582: mol_type = genomic DNA
ttgacaggtcaactagttcagtatggacgacaccgccagcgcagaagctacgcacgcataagcgaagtgttagaattaccaaatctcattgaaattcaaacctcttcttatcagtggtttcttgatgagggtcttagagagatgtttcaagatatatccccaattgaggattttactggtaacctttctcttgaattcattgattacagcctaggggatcctaagtatcctgtagcagaatcaaaagaacgtgatgtaacttactctgctccactaagagtaaaagttcgtttaattaacaaagaaactggagaagtaaaagaccaagatgtgtttatgggtgatttcccaatcatgacagacacaggtacttttatcattaatggtgcggaacgtgtaatcgtttctcagttagtacgttctccaagtgtatatttcagtggtaaagtagacaaaaacggtaaaaaaggttttactgcgactgtcattccaaaccgtggcgcatggttagaatacgaaactgatgcgaaggatgtagtctatgtacgcatcgatcgcacacgtaagttgccggttacggttcttttgcgtgctctcggcttcagctctgatcaagagattcttgacctcattggcgagaatgaatacttacgcaacacgttggaaaaagacaatacagagaatgctgataaagcacttctcgaaatctacgagcgtcttcgtcctggagagccgccaactgttgaaaatgcgaaaagcttgctagactctcgcttctttgatccgaagagatatgacttagcaaatgttggacgctacaagattaataagaagcttcatattaaaaatagactattcaatcaaaaattggctgaaacgctagttgatcctgaaacaggtgaaatcctagcagaaaaaggtcaaattttagatagaagagtgcttgataaagttcttccatacttagaaaacggcatcggatttagaaagctttatccaaacggtggcgtagtagaggatgaagtagaacttcaatctatcaagatttatgcaccaactgatcaagaaggcgagcaagtgatcaacgtgattggtaatgcatatgtagaggaagctgtgaagaatatcacgccttctgacatcattgcttcaatcagttacttctttaacctgcttcatggagtaggcgacacagatgatatcgatcaccttggtaaccgtcgtctgcgttctgtaggtgaacttctgcaaaaccaattccgtattggtttaagcagaatggagcgtgttgttcgtgaaagaatgtcgattcaagacacgaacacgatcacacctcagcagctgatcaacatccgtcctgtgatcgcttctatcaaagagttctttggtagctctcagctttctcagttcatggatcaaacaaacccgcttgctgaattgacacacaaacgtcgtctatcagcgcttggaccgggtggtttgacacgtgagcgtgcaggaatggaagttcgtgacgttcactattctcactatggtcgtatgtgtccgattgaaacaccagagggtccaaacattggtttgatcaactctctatcttcatttgcgaaagtgaaccgcttcggatttatcgaaacaccttaccgtcgggttgatcctgaaacaggtaaagtgacgccgagaatcgattacttaacggctgatgaagaggataactacgtagtagcacaagcgaacgctatattaggtgaagatggttcgtttattgatgataatatcattgctcgtttcagaggggaaaacaccgttgttcctcgaaaccgcgttgactacatggacgtttcgccgaagcaggttgtttctgcagcgacagcatgtatcccattcttagaaaacgatgactctaaccgtgctctaatgggagcgaacatgcaacgtcaggctgtgcctttgatgcagccggaatcaccgattgttggtacaggtatggagtatgtatcaggtaaagactctggtgctgctgtgatctgccgttacccaggtgttgtagaacgtgttgaagcgaagaatatttgggttcgccgttatgaagacgttgacggacaacaagtcaaaggaaacctagacaaatacagcttgctgaaatttgtccgctctaaccaagggacttgctacaaccagcgcccaattgtaagtgttggagatgaagtcgtcaaaggagaaatccttgcagacggtccttctatggaaaaaggtgaattggctctaggacgtaacgtcatggtcggcttcatgacttgggacggttacaactatgaggatgcgatcattatgagtgagcgccttgtaaaagatgacgtctacacttctattcatattgaagaatatgaatcagaagctcgtgatacaaagcttggaccagaagaaattacgcgtgatattccaaacgttggggaagatgctttacgcaaccttgacgagcgtggaatcatccgtattggtgcagaagtaaaagacggagaccttcttgtcgggaaagtaacgcctaaaggtgtaacagaactaacagctgaagaacgtctattacatgcaatcttcggtgaaaaggctcgtgaagtacgtgatacgtctctacgtgtaccacacggcggcggcggaatcatccacgatgtcaaagtctttaaccgtgaagatggagatgaattaccaccaggtgttaaccagttagtccgtgtatacatcgttcagaagcgtaaaatttctgaaggtgacaaaatggccggacgacatggtaacaaaggggttatctccaagatccttccagaagaagatatgccgtatcttccagatggaacaccgattgatatcatgttaaaccctctaggggtaccatctcgtatgaatatcggtcaggtacttgagcttcatatgggtatggctgcacgttacctaggcatccacattgcgtcaccagtatttgatggtgctcgtgaggaagatgtttgggaaacgcttgaagaagcaggtatgtcccgtgatgcgaaaacagtcctttatgacggtcgaactggtgaaccattcgacaaccgtgtatctgttggaatcatgtatatgatcaaactggctcacatggttgacgataaacttcacgcacgttcaactggaccatactcacttgttacgcaacagccactgggcggtaaagcacagtttggtggacagcgtttcggagagatggaagtatgggcacttgaagcttacggtgcagcatatacacttcaagaaatcttaactgtaaaatcggatgacgttgtgggtcgtgtgaaaacatacgaagcgatcgtcaaaggggataacgtacctgaaccaggtgtccctgaatcattcaaagtattaattaaagaacttcaaagtttaggtatggatgtgaaaattctatctggcgatgaagaagagatagaaatgagagatttagaagacgatgaggaaacgaagaaagcagacggattagcgttatctaatgacgaagatgctgcagacctcgcgcctgtcgatcttgaacgtgacgcagtcacaaaagaatag

SEQ ID NO: 47 - DNA, 1191 bp, Bacillus altitudinis
  source 1..1191: mol_type = genomic DNA
gtgaagaacaaatggtttgcctattttattggcagagtggaagtggagataagaggaagcggtattgagcggctaatcaatgagtgcacgagacaggggatcacaatttttcaagtgagccgccgtcaagacagcgtgcgcttatttattcgcctctcagatgtacatgcctttagaaaagtgcgcagacatcatgaggtgaaatgttcgtttcatcaaaagaaagggttcccgtttcttcttctatggtcgagaagaaatattggcttcaccctcgggatggcttttttcctagtgacgatattggctctttcaaatatggtgtggaaaattgagattaaaggtgcgaatccagaaacagaacaccaaatgagaaagcatctggacgaaataggggtgcaaaaagggcgttttcagtttctcatggggacccctgaaaaaatacaaaaatcattgacgaccaatattcagagcattacatgggtcggagttgaactgaacggaacgacgtttcaaatgaaagtggtcgaaaaaaatgaacctgaaaaggagaaatatacaagtcctcagcacatcgttgccaagaaaaaggcggtcatcacgagaatgtatgtagaaaagggggaaccgcttgcccaggtcgatgagcatgtgaaaaaagggcagatgctcgtctcaggtttaatcgggagtgaagatcagaaaaaaacggtcggagccaaagcgaaaatctatggtgaaacatggtaccgatctgaagtttctgtccctcttcgaacatcttttgatgtctttacgggtaaaatgaagacaaagcacaagctctccttgtttggaggctccatcccattttggggattttcctttaaaaaagatgattttcagcagccgaaaatagaaacagaagttcatccgcttcattttttgaatatgcaattgccgttctcctatgaaaaggaaatcacacgagaaagtgaaaaaataaatcgagaatacacaaataaagaagcggttcaagcagggattaaaatgggtaaaaaagaattagaagaaaagctaggtcaaacaggtgaggtgaaaagtgaaaaagttttgcacgagacaacagggaatggtaaagttaagttaatcatcctttaccaagtaatagaagatattgttcaaccaacacctattgttcagggagactag

SEQ ID NO: 48 - DNA, 1550 bp, Bacillus subtilis
  source 1..1550: mol_type = genomic DNA
ttatcggagagtttgatcctggctcaggacgaacgctggcggcgtgcctaatacatgcaagtcgagcggacagatgggagcttgctccctgatgttagcggcggacgggtgagtaacacgtgggtaacctgcctgtaagactgggataactccgggaaaccggggctaataccggatggttgtttgaaccgcatggttcaaacataaaaggtggcttcggctaccacttacagatggacccgcggcgcattagctagttggtgaggtaacggctcaccaaggcaacgatgcgtagccgacctgagagggtgatcggccacactgggactgagacacggcccagactcctacgggaggcagcagtagggaatcttccgcaatggacgaaagtctgacggagcaacgccgcgtgagtgatgaaggttttcggatcgtaaagctctgttgttagggaagaacaagtaccgttcgaatagggcggtaccttgacggtacctaaccagaaagccacggctaactacgtgccagcagccgcggtaatacgtaggtggcaagcgttgtccggaattattgggcgtaaagggctcgcaggcggtttcttaagtctgatgtgaaagcccccggctcaaccggggagggtcattggaaactggggaacttgagtgcagaagaggagagtggaattccacgtgtagcggtgaaatgcgtagagatgtggaggaacaccagtggcgaaggcgactctctggtctgtaactgacgctgaggagcgaaagcgtggggagcgaacaggattagataccctggtagtccacgccgtaaacgatgagtgctaagtgttagggggtttccgccccttagtgctgcagctaacgcattaagcactccgcctggggagtacggtcgcaagactgaaactcaaaggaattgacgggggcccgcacaagcggtggagcatgtggtttaattcgaagcaacgcgaagaaccttaccaggtcttgacatcctctgacaatcctagagataggacgtccccttcgggggcagagtgacaggtggtgcatggttgtcgtcagctcgtgtcgtgagatgttgggttaagtcccgcaacgagcgcaacccttgatcttagttgccagcattcagttgggcactctaaggtgactgccggtgacaaaccggaggaaggtggggatgacgtcaaatcatcatgccccttatgacctgggctacacacgtgctacaatggacagaacaaagggcagcgaaaccgcgaggttaagccaatcccacaaatctgttctcagttcggatcgcagtctgcaactcgactgcgtgaagctggaatcgctagtaatcgcggatcagcatgccgcggtgaatacgttcccgggccttgtacacaccgcccgtcacaccacgagagtttgtaacacccgaagtcggtgaggtaaccttttaggagccagccgccgaaggtgggacagatgattggggtgaagtcgtaacaaggtagccgtatcggaaggtgcggctggatcacctccttt

SEQ ID NO: 49 - DNA, 1632 bp, Bacillus subtilis
  source 1..1632: mol_type = genomic DNA
atggcaaaagaaattaagtttagtgaagaagctcgccgcgcaatgcttcgtggtgtcgatgcacttgctgatgctgttaaagtaactttaggaccaaaaggacgcaacgtggttctagagaaaaaattcggttctccgttaatcacaaatgacggtgtaacaatcgctaaagaaatcgagctagaagacgcgtttgaaaacatgggtgctaagcttgttgctgaagtagccagcaaaacaaacgacgttgccggtgacggtacaacaactgcaacagttcttgcgcaagcaatgatccgtgaaggccttaaaaacgtaacagcaggcgctaaccctgtaggcgtgcgtaaagggatggaacaagctgtatcggttgcgatcgaaaacttaaaagaaatttctaagccaatcgaaggcaaagagtctatcgctcaggttgctgcgatctctgctgctgatgaggaagtcggaagccttatcgctgaagcaatggagcgcgtaggaaacgacggcgttatcacaatcgaagagtctaaaggcttcacaactgagcttgaagttgttgaaggtatgcaattcgaccgcggatatgcgtctccttacatggtaactgactctgataagatggaagcggttcttgacaatccttacatcttaatcacagacaaaaaaatcacaaacattcaagaaatccttcctgtgcttgagcaggttgttcagcaaggcaaaccattgcttctgatcgctgaggatgttgaaggcgaagcacttgctacacttgttgtgaacaaacttcgcggcacattcaacgcagtggctgttaaagctcctggcttcggtgatcgccgtaaagcaatgcttgaagacatcgctgtccttactggcggagaagtcatcacagaagatcttggccttgacctgaaatctactcaaatcgctcaattgggacgcgcttctaaagttgtcgttactaaagaaaacacaacaatcgttgaaggcgctggcgaaacagacaaaatttctgcccgtgtgactcaaatccgcgctcaagtggaagaaacaacttctgaattcgacagagaaaaattacaagagcgtcttgcgaaacttgctggcggcgtagctgtcatcaaagtcggcgctgcgactgaaactgaactgaaagagcgtaaacttcgcatcgaagacgccttgaactcaactcgcgcagctgttgaagaaggcatcgtatccggtggtggtacagcgcttgtaaacgtatataacaaagtcgctgcagttgaagctgaaggcgatgctcaaacaggtatcaacatcgtgcttcgcgcgcttgaagagccaatccgtcaaatcgcacataacgctggtcttgaaggatctgtcatcgttgagcgcctcaaaaacgaagaaatcggcgtaggcttcaacgctgcaactggcgaatgggtaaacatgatcgaaaaaggtatcgttgacccaacgaaagttacacgctcagctcttcaaaacgctgcgtctgtagctgcaatgttcttaacaactgaagccgttgtcgctgacaagccagaagaaaacactggcggcggaatgcctgacatgggcggcatgggcggtatgggtggtatgatgtaa

SEQ ID NO: 50 - DNA, 1923 bp, Bacillus subtilis
  source 1..1923: mol_type = genomic DNA
gtggctatggaacagcagcaaaacagttatgatgaaaatcagatacaggtactagaaggattggaagctgttcgtaaaagaccggggatgtatatcggttcgacaaacagcaaaggccttcaccacctggtatgggagattgtcgacaatagtattgacgaagccctcgccggttattgtacggatatcaatatccaaatcgaaaaagacaacagtatcacggttgtagataatggccgcggtattccagtcggtattcatgaaaaaatgggccgtcctgcggtagaagtcattatgacggtgcttcatgccggaggaaaatttgacggaagcggctataaagtatccggaggattacacggtgtaggtgcttcggtcgtaaacgcactatccacagagcttgatgtgacggttcaccgtgacggtaaaattcatcgccaaacctataagcgcggagttccggttacagaccttgaaatcattggcgaaacggatcatacaggaacgacgacacattttgtcccggaccctgaaattttctcagaaacaaccgagtatgattatgatctgcttgccaaccgcgtgcgtgaattagcctttttaacaaagggtgtaaacatcacgattgaagataaacgtgaaggacaagagcgcaaaaatgaataccattacgaaggcggaattaaaagttatgtagagtatttaaaccgctctaaagaggttgtccatgaagagccgatttacattgaaggcgaaaaggacggcattacggttgaagtggctttgcaatacaatgacagctacacaagcaacatttactcgtttacaaacaacattaacacgtacgaaggcggtacccatgaagctggcttcaaaacgggcctgactcgtgttatcaacgattacgccagaaaaaaagggcttattaaagaaaatgatccaaacctaagcggagatgacgtaagggaagggctgacagcgattatttcaatcaaacaccctgatccgcagtttgagggccaaacgaaaacaaagctgggcaactcagaagcacggacaatcaccgatacgttattttctacagcgatggaaacatttatgctggaaaatccagatgcagccaaaaaaattgtcgataaaggcttaatggcggcaagagcaagaatggctgcgaaaaaagcccgtgaactaacacgtcgtaagagtgctttggaaatttcaaacttgcccggtaagttagcggactgctcttcaaaagatccgagcatttccgagttatatatcgtagagggtgactctgccggaggatctgctaaacaaggacgcgacagacatttccaagccattttgccgcttagaggtaaaatcctaaacgttgaaaaggccagactggataaaatcctttctaacaacgaagttcgctctatgatcacagcgctcggcacaggtattggggaagacttcaaccttgagaaagcccgttaccacaaagttgtcattatgacagatgccgatgttgacggcgcgcacatcagaacactgctgttaacgttcttttacagatatatgcgccaaattatcgaaaatggctacgtgtacattgcacagccgccgctctacaaggttcaacaggggaaacgtgttgaatatgcgtacaatgacaaggagcttgaagagctgttaaaaactcttcctcaaacgcctaagcctggactgcagcgttacaaaggtcttggtgaaatgaatgccacccagctatgggagacaaccatggatcctagctccagaacacttcttcaggtaactcttgaagatgcaatggatgcggacgagacttttgaaatgcttatgggcgacaaagtagaaccgcgccgaaacttcatagaagcgaatgcgagatacgttaaaaatcttgacatctaa

SEQ ID NO: 51 - DNA, 3582 bp, Bacillus subtilis
  source 1..3582: mol_type = genomic DNA
ttgacaggtcaactagttcagtatggacgacaccgccagcgcagaagctatgctcgcattagcgaagtgttagaattaccaaatctcattgaaattcaaacctcttcttatcagtggtttcttgatgagggtcttagagagatgtttcaagacatatcaccaattgaggatttcactggtaacctctctcttgagttcattgattatagtttaggtgagcctaaatatcctgtagaggaatcaaaagaacgtgatgtgacttactcagctccgctaagagtgaaggttcgtttaattaacaaagaaactggagaggtaaaagaccaagatgtcttcatgggtgatttccctattatgacagatacaggtacttttatcattaacggtgcggaacgtgttatcgtttcccagcttgttcggtctccaagtgtatatttcagtggtaaagtagacaaaaacggtaaaaaaggttttaccgcaactgtcattccaaaccgtggcgcatggttagaatacgaaactgatgcgaaagatgttgtttatgtccgcattgatcgcacacgtaagttgccggttacggttcttttgcgtgctctcggcttcggctccgatcaagagattcttgatctcataggagaaaacgaatacctgcgaaatacgcttgataaagataacacagaaaacagcgacaaagcgttgctggaaatttacgagcgtctccgtcctggagagccgcctacagtagaaaatgcgaaaagcttgcttgattctcgtttctttgatccgaaacgatacgatcttgccaatgtaggacgctataaaattaataaaaaacttcatattaagaatcgcctcttcaatcagagacttgctgaaacgcttgttgatcctgaaacaggagaaatccttgctgaaaaaggtcagattcttgatagaagaacacttgataaagtactgccatacttagaaaacggaatcggtttcagaaagctgtatccgaatggcggcgttgttgaagatgaagtgactcttcaatcaattaaaatctttgctccgactgatcaagaaggagaacaggttattaatgtaatcggcaatgcttacatcgaagaagagattaaaaacatcacgcctgctgatattatttcttcaatcagctacttcttcaacctgctgcacggagtaggcgacacagatgatatcgatcatcttggaaaccgccgtttacgttctgtaggcgagcttctccagaatcaattccgtatcggtttaagccgtatggagcgtgtggttcgtgagagaatgtcaattcaagatacgaatacaattacgcctcagcagctgatcaatattcgtcctgttattgcgtccattaaagagttctttggaagctcacagctttctcaattcatggatcagacgaacccgcttgctgaattaacgcacaagcgtcgtctgtcagcattaggaccgggcggattgacacgtgagcgtgccggaatggaagtgcgtgacgttcactactcccactatggccgtatgtgtccgattgaaacgcctgagggcccgaacatcggtttgatcaactcactatcatcttatgcaaaagtaaaccgttttggctttattgaaacgccatatcgccgcgttgaccctgaaacagggaaggtaacgggcagaatcgattacttaactgctgatgaagaggataactatgttgtcgctcaagcgaatgctcgtcttgatgacgaaggcgcctttattgatgacagcatcgtagctcgtttccgcggggagaacaccgttgtttccagaaatcgtgtagactacatggatgtatcgcctaagcaggttgtatctgctgcgacagcatgtatcccgttcttagaaaacgatgactccaaccgtgccctcatgggagcgaacatgcagcgtcaggctgtgcctttgatgcagccggaagcgccatttgttggaactggtatggaatacgtatcaggaaaagactctggtgccgctgttatttgtaaacaccctggtatcgttgaacgcgtagaagcgaaaaacgtttgggttcgccgttatgaagaagtagacggtcaaaaagtaaaaggaaacctggataaatacagcctgctgaaatttgtccgctctaaccaaggtacgtgctacaaccagcgtccgatcgtaagtgtcggcgatgaagtggtaaaaggagaaatccttgctgacggtccttctatggagcttggtgaacttgcacttggccgtaacgtaatggtcggcttcatgacatgggatggctacaactatgaggatgccatcatcatgagtgaacgcctagtgaaggatgatgtttatacatctatccacattgaagaatacgaatcagaagcacgtgatacgaaacttggacctgaagaaatcactcgcgatattccaaacgtcggtgaagatgcgcttcgcaatcttgatgaccgcggaatcatccgtattggggcagaagtaaaagacggagatcttcttgttggtaaagtaacgcctaaaggcgtaactgaactgactgcagaagaacgccttcttcacgccatctttggcgagaaagcccgcgaggttcgtgatacttctcttcgtgtgcctcacggcggcggcggaattatccatgacgttaaagtcttcaaccgtgaagacggagacgaacttcctccaggtgttaaccagttagtacgcgtatatatcgttcagaaacgtaagatttctgaaggggataaaatggccggtcgtcacggtaacaaaggtgttatctctaagattcttcctgaagaggatatgccttaccttcctgacggcacaccaattgatatcatgcttaacccgctgggcgtaccatcacgtatgaacatcgggcaggtattggaacttcacatgggtatggccgctcgttaccttggcattcacattgcatctcctgtatttgacggagcgcgagaagaggatgtctgggaaacacttgaagaagccggcatgtctcgtgacgccaaaacagtgctttacgacggacgtactggagagccgtttgataaccgtgtatctgtcggtatcatgtacatgatcaaactagctcacatggttgacgataaacttcatgcacgctctacaggcccttactcacttgttacgcagcagcctcttggcggtaaagcgcaatttggcggacagcgttttggtgagatggaggtttgggcacttgaagcttacggtgcggcttacactcttcaagaaattctgactgttaagtctgatgacgtggttggacgtgtgaaaacatacgaagccatcgttaaaggcgacaatgttcctgaaccaggtgttccggaatcattcaaagtattaatcaaagaacttcaaagcttaggtatggatgtcaaaatcctttctggtgatgaagaagaaatagaaatgagagatttagaagacgaagaagatgcgaaacaagctgacggcctggcattatcaggtgatgaagagccggaagaaacagcatctgcagacgttgaacgcgatgtagtaacaaaagaataa

SEQ ID NO: 52 - DNA, 1197 bp, Bacillus subtilis
  source 1..1197: mol_type = genomic DNA
gtgaaaaataaatggctgtcttttttttcgggtaaggtccagcttgaattgacgggaagagggattgagcggctccttaatgaatgcacaagacaggggattccggtctttcatgtcaaaaaaaagaaagaagccgtatcgttatatatacagcttcaggatgtacatgcctttcggcgggtgagaagtaaatttaaatgtaaagcccgatttatcaatcggaagggttttcccttcctgttgctgaaatcaaagctgaatatagggtttacgatcggttttgcgatttttttcatccttttgtttctgctttccaatatggtgtggaaaattgatgtgacaggcgctaagcctgaaacagagcatcaaatgaggcagcatcttaatgaaatcggcgttaaaaagggccgtctgcagtttttaatgatgtcgcccgaaaaaatacagaaatcattaaccaatggaatagacaatatcacttgggtcggtgttgatctgaaggggacgaccattcacatgaaagtcgtagagaaaaatgagcccgaaaaagaaaagtatgttagcccgcgcaatattgtcgccaaaaagaaagcaaccattacgagaatgtttgtgcaaaaaggacagcccatggctgccatccacgatcatgttgaaaaggggcagctgcttgtttcgggactgatcggcagcgaagaccatcagcaggaagtcgcctcaaaagcagaaatttacggagaaacctggtatagatcagaagtgactgtcccgcttgaaacattatttaacgtctatacgggcaaagtaaggacaaagcacaagctttcttttggctcgttggcaatcccgatctgggggatgacgtttaaaaaagaggaattgaagcatccaaaaacagaacaagaaaaacattcgcttcattttctcggatttaagctccctgtatcttatgtcaaagagcaaacgagagaaagtgaagaggctttgcgaaaatatacgaaagaagaagcagttcaagaaggcattaaattgggtaaacaggatgtagaggataaaataggcgaaaacggcgaggtgaaaagtgaaaaagttttgcaccagactgttgagaatggtaaagtaaagttgattattctctaccaagttatagaagatatcgttcaaaccacacctattgtcagggagactgaagaatga